European Patent Specification EP 3 600 407 B1, published January 29, 2025. Title: Improved antigen binding receptors. Applicant: F. Hoffmann-La Roche Ltd. The sequence listing filed with the application follows.

SEQUENCE LISTING (130 sequences)

SEQ ID NO: 1 - protein, 5 aa, Artificial sequence
  Anti-P329G CDR H1 Kabat
RYWMN

SEQ ID NO: 2 - protein, 17 aa, Artificial sequence
  Anti-P329G CDR H2 Kabat
EITPDSSTINYTPSLKD

SEQ ID NO: 3 - protein, 10 aa, Artificial sequence
  Anti-P329G CDR H3 Kabat
PYDYGAWFAS

SEQ ID NO: 4 - protein, 14 aa, Artificial sequence
  Anti-P329G CDR L1 Kabat
RSSTGAVTTSNYAN

SEQ ID NO: 5 - protein, 7 aa, Artificial sequence
  Anti-P329G CDR L2 Kabat
GTNKRAP

SEQ ID NO: 6 - protein, 9 aa, Artificial sequence
  Anti-P329G CDR L3 Kabat
ALWYSNHWV

SEQ ID NO: 7 - protein, 433 aa, Artificial sequence
  Anti-P329G-ds-scFv-CD28ATM-CD28CSD-CD3zSSD fusion pETR17096
EVKLLESGGGLVQPGGSLKLSCAASGFDFSRYWMNWVRQAPGKCLEWIGEITPDSSTINYTPSLKDKFIISRDNAKNTLYLQMIKVRSEDTALYYCVRPYDYGAWFASWGQGTLVTVSAGGGGSGGGGSGGGGSGGGGSQAVVTQESALTTSPGETVTLTCRSSTGAVTTSNYANWVQEKPDHLFTGLIGGTNKRAPGVPARFSGSLIGDKAALTITGAQTEDEAIYFCALWYSNHWVFGCGTKLTVLGGGGSFWVLVVVGGVLACYSLLVTVAFIIFWVRSKRSRLLHSDYMNMTPRRPGPTRKHYQPYAPPRDFAAYRSRVKFSRSADAPAYQQGQNQLYNELNLGRREEYDVLDKRRGRDPEMGGKPRRKNPQEGLYNELQKDKMAEAYSEIGMKGERRRGKGHDGLYQGLSTATKDTYDALHMQALPPR

SEQ ID NO: 8 - protein, 119 aa, Artificial sequence
  Anti-P329G-ds VH
EVKLLESGGGLVQPGGSLKLSCAASGFDFSRYWMNWVRQAPGKCLEWIGEITPDSSTINYTPSLKDKFIISRDNAKNTLYLQMIKVRSEDTALYYCVRPYDYGAWFASWGQGTLVTVSA

SEQ ID NO: 9 - protein, 109 aa, Artificial sequence
  Anti-P329G-ds VL
QAVVTQESALTTSPGETVTLTCRSSTGAVTTSNYANWVQEKPDHLFTGLIGGTNKRAPGVPARFSGSLIGDKAALTITGAQTEDEAIYFCALWYSNHWVFGCGTKLTVL

SEQ ID NO: 10 - protein, 248 aa, Artificial sequence
  Anti-P329G-ds-scFv
EVKLLESGGGLVQPGGSLKLSCAASGFDFSRYWMNWVRQAPGKCLEWIGEITPDSSTINYTPSLKDKFIISRDNAKNTLYLQMIKVRSEDTALYYCVRPYDYGAWFASWGQGTLVTVSAGGGGSGGGGSGGGGSGGGGSQAVVTQESALTTSPGETVTLTCRSSTGAVTTSNYANWVQEKPDHLFTGLIGGTNKRAPGVPARFSGSLIGDKAALTITGAQTEDEAIYFCALWYSNHWVFGCGTKLTVL

SEQ ID NO: 11 - protein, 27 aa, Artificial sequence
  CD28ATM
FWVLVVVGGVLACYSLLVTVAFIIFWV

SEQ ID NO: 12 - protein, 41 aa, Artificial sequence
  CD28CSD
RSKRSRLLHSDYMNMTPRRPGPTRKHYQPYAPPRDFAAYRS

SEQ ID NO: 13 - protein, 112 aa, Artificial sequence
  CD3zSSD
RVKFSRSADAPAYQQGQNQLYNELNLGRREEYDVLDKRRGRDPEMGGKPRRKNPQEGLYNELQKDKMAEAYSEIGMKGERRRGKGHDGLYQGLSTATKDTYDALHMQALPPR

SEQ ID NO: 14 - protein, 180 aa, Artificial sequence
  CD28ATM-CD28-CD3z
FWVLVVVGGVLACYSLLVTVAFIIFWVRSKRSRLLHSDYMNMTPRRPGPTRKHYQPYAPPRDFAAYRSRVKFSRSADAPAYQQGQNQLYNELNLGRREEYDVLDKRRGRDPEMGGKPRRKNPQEGLYNELQKDKMAEAYSEIGMKGERRRGKGHDGLYQGLSTATKDTYDALHMQALPPR

SEQ ID NO: 15 - protein, 238 aa, Artificial sequence
  eGFP
VSKGEELFTGVVPILVELDGDVNGHKFSVSGEGEGDATYGKLTLKFICTTGKLPVPWPTLVTTLTYGVQCFSRYPDHMKQHDFFKSAMPEGYVQERTIFFKDDGNYKTRAEVKFEGDTLVNRIELKGIDFKEDGNILGHKLEYNYNSHNVYIMADKQKNGIKVNFKIRHNIEDGSVQLADHYQQNTPIGDGPVLLPDNHYLSTQSALSKDPNEKRDHMVLLEFVTAAGITLGMDELYK

SEQ ID NO: 16 - protein, 20 aa, Artificial sequence
  (G4S)4 linker
GGGGSGGGGSGGGGSGGGGS

SEQ ID NO: 17 - protein, 5 aa, Artificial sequence
  G4S linker
GGGGS

SEQ ID NO: 18 - protein, 19 aa, Artificial sequence
  T2A linker
GEGRGSLLTCGDVEENPGP

SEQ ID NO: 19 - DNA, 1356 bp, Artificial sequence
  Anti-P329G-ds-scFv-CD28ATM-CD28CSD-CD3zSSD fusion pETR17096
atgggatggagctgtatcatcctcttcttggtagcaacagctaccggtgtgcattccgaggtgaagctgctggagagcggcggcggcctggtgcagcccggcggcagcctgaagctgagctgcgccgccagcggcttcgacttcagcaggtactggatgaactgggtgaggcaggcccccggcaagtgtctggagtggatcggcgagatcacccccgacagcagcaccatcaactacacccccagcctgaaggacaagttcatcatcagcagggacaacgccaagaacaccctgtacctgcagatgatcaaggtgaggagcgaggacaccgccctgtactactgcgtgaggccctacgactacggcgcctggttcgccagctggggccagggcaccctggtgaccgtgagcgccggagggggcggaagtggtggcgggggaagcggcgggggtggcagcggagggggcggatctcaggccgtggtgacccaggagagcgccctgaccaccagccccggcgagaccgtgaccctgacctgcaggagcagcaccggcgccgtgaccaccagcaactacgccaactgggtgcaggagaagcccgaccacctgttcaccggcctgatcggcggcaccaacaagagggcccccggcgtgcccgccaggttcagcggcagcctgatcggcgacaaggccgccctgaccatcaccggcgcccagaccgaggacgaggccatctacttctgcgccctgtggtacagcaaccactgggtgttcggctgtggcaccaagctgaccgtgctgggagggggcggatccttctgggtgctggtggtggtgggcggcgtgctggcctgctacagcctgctggtgaccgtggccttcatcatcttctgggtgaggagcaagaggagcaggctgctgcacagcgactacatgaacatgacccccaggaggcccggccccaccaggaagcactaccagccctacgccccccccagggacttcgccgcctacaggagcagggtgaagttcagcaggagcgccgacgcccccgcctaccagcagggccagaaccagctgtataacgagctgaacctgggcaggagggaggagtacgacgtgctggacaagaggaggggcagggaccccgagatgggcggcaagcccaggaggaagaacccccaggagggcctgtataacgagctgcagaaggacaagatggccgaggcctacagcgagatcggcatgaagggcgagaggaggaggggcaagggccacgacggcctgtaccagggcctgagcaccgccaccaaggacacctacgacgccctgcacatgcaggccctgccccccagg

SEQ ID NO: 20 - DNA, 357 bp, Artificial sequence
  Anti-P329G-ds VH
gaggtgaagctgctggagagcggcggcggcctggtgcagcccggcggcagcctgaagctgagctgcgccgccagcggcttcgacttcagcaggtactggatgaactgggtgaggcaggcccccggcaagtgtctggagtggatcggcgagatcacccccgacagcagcaccatcaactacacccccagcctgaaggacaagttcatcatcagcagggacaacgccaagaacaccctgtacctgcagatgatcaaggtgaggagcgaggacaccgccctgtactactgcgtgaggccctacgactacggcgcctggttcgccagctggggccagggcaccctggtgaccgtgagcgcc

SEQ ID NO: 21 - DNA, 327 bp, Artificial sequence
  Anti-P329G-ds VL
caggccgtggtgacccaggagagcgccctgaccaccagccccggcgagaccgtgaccctgacctgcaggagcagcaccggcgccgtgaccaccagcaactacgccaactgggtgcaggagaagcccgaccacctgttcaccggcctgatcggcggcaccaacaagagggcccccggcgtgcccgccaggttcagcggcagcctgatcggcgacaaggccgccctgaccatcaccggcgcccagaccgaggacgaggccatctacttctgcgccctgtggtacagcaaccactgggtgttcggctgtggcaccaagctgaccgtgctg

SEQ ID NO: 22 - DNA, 799 bp, Artificial sequence
  Anti-P329G-ds-scFv
atgggatggagctgtatcatcctcttcttggtagcaacagctaccggtgtgcattccgaggtgaagctgctggagagcggcggcggcctggtgcagcccggcggcagcctgaagctgagctgcgccgccagcggcttcgacttcagcaggtactggatgaactgggtgaggcaggcccccggcaagtgtctggagtggatcggcgagatcacccccgacagcagcaccatcaactacacccccagcctgaaggacaagttcatcatcagcagggacaacgccaagaacaccctgtacctgcagatgatcaaggtgaggagcgaggacaccgccctgtactactgcgtgaggccctacgactacggcgcctggttcgccagctggggccagggcaccctggtgaccgtgagcgccggagggggcggaagtggtggcgggggaagcggcgggggtggcagcggagggggcggatctcaggccgtggtgacccaggagagcgccctgaccaccagccccggcgagaccgtgaccctgacctgcaggagcagcaccggcgccgtgaccaccagcaactacgccaactgggtgcaggagaagcccgaccacctgttcaccggcctgatcggcggcaccaacaagagggcccccggcgtgcccgccaggttcagcggcagcctgatcggcgacaaggccgccctgaccatcaccggcgcccagaccgaggacgaggccatctacttctgcgccctgtggtacagcaaccactgggtgttcggctgtggcaccaagctgaccgtgc

SEQ ID NO: 23 - DNA, 647 bp, Artificial sequence
  IRES EV71, internal ribosomal entry side
cccgaagtaacttagaagctgtaaatcaacgatcaatagcaggtgtggcacaccagtcataccttgatcaagcacttctgtttccccggactgagtatcaataggctgctcgcgcggctgaaggagaaaacgttcgttacccgaccaactacttcgagaagcttagtaccaccatgaacgaggcagggtgtttcgctcagcacaaccccagtgtagatcaggctgatgagtcactgcaacccccatgggcgaccatggcagtggctgcgttggcggcctgcccatggagaaatccatgggacgctctaattctgacatggtgtgaagtgcctattgagctaactggtagtcctccggcccctgattgcggctaatcctaactgcggagcacatgctcacaaaccagtgggtggtgtgtcgtaacgggcaactctgcagcggaaccgactactttgggtgtccgtgtttccttttattcctatattggctgcttatggtgacaatcaaaaagttgttaccatatagctattggattggccatccggtgtgcaacagggcaactgtttacctatttattggttttgtaccattatcactgaagtctgtgatcactctcaaattcattttgaccctcaacacaatcaaac

SEQ ID NO: 24 - DNA, 81 bp, Artificial sequence
  CD28ATM
ttttgggtgctggtggtggttggtggagtcctggcttgctatagcttgctagtaacagtggcctttattattttctgggtg

SEQ ID NO: 25 - DNA, 123 bp, Artificial sequence
  CD28CSD
aggagtaagaggagcaggctcctgcacagtgactacatgaacatgactccccgccgccccgggcccacccgcaagcattaccagccctatgccccaccacgcgacttcgcagcctatcgctcc

SEQ ID NO: 26 - DNA, 336 bp, Artificial sequence
  CD3z SSD
agagtgaagttcagcaggagcgcagacgcccccgcgtaccagcagggccagaaccagctctataacgagctcaatctaggacgaagagaggagtacgatgttttggacaagagacgtggccgggaccctgagatggggggaaagccgagaaggaagaaccctcaggaaggcctgtacaatgaactgcagaaagataagatggcggaggcctacagtgagattgggatgaaaggcgagcgccggaggggcaaggggcacgatggcctttaccagggtctcagtacagccaccaaggacacctacgacgcccttcacatgcaggccctgccccctcgc

SEQ ID NO: 27 - DNA, 540 bp, Artificial sequence
  CD28ATM-CD28-CD3z
ttctgggtgctggtggtggtgggcggcgtgctggcctgctacagcctgctggtgaccgtggccttcatcatcttctgggtgaggagcaagaggagcaggctgctgcacagcgactacatgaacatgacccccaggaggcccggccccaccaggaagcactaccagccctacgccccccccagggacttcgccgcctacaggagcagggtgaagttcagcaggagcgccgacgcccccgcctaccagcagggccagaaccagctgtataacgagctgaacctgggcaggagggaggagtacgacgtgctggacaagaggaggggcagggaccccgagatgggcggcaagcccaggaggaagaacccccaggagggcctgtataacgagctgcagaaggacaagatggccgaggcctacagcgagatcggcatgaagggcgagaggaggaggggcaagggccacgacggcctgtaccagggcctgagcaccgccaccaaggacacctacgacgccctgcacatgcaggccctgccccccagg

SEQ ID NO: 28 - DNA, 63 bp, Artificial sequence
  T2A element
tccggagagggcagaggaagtcttctaacatgcggtgacgtggaggagaatcccggccctagg

SEQ ID NO: 29 - DNA, 717 bp, Artificial sequence
  eGFP
gtgagcaagggcgaggagctgttcaccggggtggtgcccatcctggtcgagctggacggcgacgtaaacggccacaagttcagcgtgtccggcgagggcgagggcgatgccacctacggcaagctgaccctgaagttcatctgcaccaccggcaagctgcccgtgccctggcccaccctcgtgaccaccctgacctacggcgtgcagtgcttcagccgctaccccgaccacatgaagcagcacgacttcttcaagtccgccatgcccgaaggctacgtccaggagcgcaccatcttcttcaaggacgacggcaactacaagacccgcgccgaggtgaagttcgagggcgacaccctggtgaaccgcatcgagctgaagggcatcgacttcaaggaggacggcaacatcctggggcacaagctggagtacaactacaacagccacaacgtctatatcatggccgacaagcagaagaacggcatcaaggtgaacttcaagatccgccacaacatcgaggacggcagcgtgcagctcgccgaccactaccagcagaacacccccatcggcgacggccccgtgctgctgcccgacaaccactacctgagcacccagtccgccctgagcaaagaccccaacgagaagcgcgatcacatggtcctgctggagttcgtgaccgccgccgggatcactctcggcatggacgagctgtacaagtga

SEQ ID NO: 30 - DNA, 2136 bp, Artificial sequence
  Anti-P329G-ds-scFv-CD28ATM-CD28CSD-CD3zSSD-eGFP fusion pETR17096
atgggatggagctgtatcatcctcttcttggtagcaacagctaccggtgtgcattccgaggtgaagctgctggagagcggcggcggcctggtgcagcccggcggcagcctgaagctgagctgcgccgccagcggcttcgacttcagcaggtactggatgaactgggtgaggcaggcccccggcaagtgtctggagtggatcggcgagatcacccccgacagcagcaccatcaactacacccccagcctgaaggacaagttcatcatcagcagggacaacgccaagaacaccctgtacctgcagatgatcaaggtgaggagcgaggacaccgccctgtactactgcgtgaggccctacgactacggcgcctggttcgccagctggggccagggcaccctggtgaccgtgagcgccggagggggcggaagtggtggcgggggaagcggcgggggtggcagcggagggggcggatctcaggccgtggtgacccaggagagcgccctgaccaccagccccggcgagaccgtgaccctgacctgcaggagcagcaccggcgccgtgaccaccagcaactacgccaactgggtgcaggagaagcccgaccacctgttcaccggcctgatcggcggcaccaacaagagggcccccggcgtgcccgccaggttcagcggcagcctgatcggcgacaaggccgccctgaccatcaccggcgcccagaccgaggacgaggccatctacttctgcgccctgtggtacagcaaccactgggtgttcggctgtggcaccaagctgaccgtgctgggagggggcggatccttctgggtgctggtggtggtgggcggcgtgctggcctgctacagcctgctggtgaccgtggccttcatcatcttctgggtgaggagcaagaggagcaggctgctgcacagcgactacatgaacatgacccccaggaggcccggccccaccaggaagcactaccagccctacgccccccccagggacttcgccgcctacaggagcagggtgaagttcagcaggagcgccgacgcccccgcctaccagcagggccagaaccagctgtataacgagctgaacctgggcaggagggaggagtacgacgtgctggacaagaggaggggcagggaccccgagatgggcggcaagcccaggaggaagaacccccaggagggcctgtataacgagctgcagaaggacaagatggccgaggcctacagcgagatcggcatgaagggcgagaggaggaggggcaagggccacgacggcctgtaccagggcctgagcaccgccaccaaggacacctacgacgccctgcacatgcaggccctgccccccaggtccggagagggcagaggaagtcttctaacatgcggtgacgtggaggagaatcccggccctagggtgagcaagggcgaggagctgttcaccggggtggtgcccatcctggtcgagctggacggcgacgtaaacggccacaagttcagcgtgtccggcgagggcgagggcgatgccacctacggcaagctgaccctgaagttcatctgcaccaccggcaagctgcccgtgccctggcccaccctcgtgaccaccctgacctacggcgtgcagtgcttcagccgctaccccgaccacatgaagcagcacgacttcttcaagtccgccatgcccgaaggctacgtccaggagcgcaccatcttcttcaaggacgacggcaactacaagacccgcgccgaggtgaagttcgagggcgacaccctggtgaaccgcatcgagctgaagggcatcgacttcaaggaggacggcaacatcctggggcacaagctggagtacaactacaacagccacaacgtctatatcatggccgacaagcagaagaacggcatcaaggtgaacttcaagatccgccacaacatcgaggacggcagcgtgcagctcgccgaccactaccagcagaacacccccatcggcgacggccccgtgctgctgcccgacaaccactacctgagcacccagtccgccctgagcaaagaccccaacgagaagcgcgatcacatggtcctgctggagttcgtgaccgccgccgggatcactctcggcatggacgagctgtacaagtga

SEQ ID NO: 31 - protein, 433 aa, Artificial sequence
  Anti-P329G-scFv- CD28ATM-CD28CSD-CD3zSSD fusion
EVKLLESGGGLVQPGGSLKLSCAASGFDFSRYWMNWVRQAPGKGLEWIGEITPDSSTINYTPSLKDKFIISRDNAKNTLYLQMIKVRSEDTALYYCVRPYDYGAWFASWGQGTLVTVSAGGGGSGGGGSGGGGSGGGGSQAVVTQESALTTSPGETVTLTCRSSTGAVTTSNYANWVQEKPDHLFTGLIGGTNKRAPGVPARFSGSLIGDKAALTITGAQTEDEAIYFCALWYSNHWVFGGGTKLTVLGGGGSFWVLVVVGGVLACYSLLVTVAFIIFWVRSKRSRLLHSDYMNMTPRRPGPTRKHYQPYAPPRDFAAYRSRVKFSRSADAPAYQQGQNQLYNELNLGRREEYDVLDKRRGRDPEMGGKPRRKNPQEGLYNELQKDKMAEAYSEIGMKGERRRGKGHDGLYQGLSTATKDTYDALHMQALPPR

SEQ ID NO: 32 - protein, 119 aa, Artificial sequence
  Anti-P329G VH
EVKLLESGGGLVQPGGSLKLSCAASGFDFSRYWMNWVRQAPGKGLEWIGEITPDSSTINYTPSLKDKFIISRDNAKNTLYLQMIKVRSEDTALYYCVRPYDYGAWFASWGQGTLVTVSA

SEQ ID NO: 33 - protein, 109 aa, Artificial sequence
  Anti-P329G VL
QAVVTQESALTTSPGETVTLTCRSSTGAVTTSNYANWVQEKPDHLFTGLIGGTNKRAPGVPARFSGSLIGDKAALTITGAQTEDEAIYFCALWYSNHWVFGGGTKLTVL

SEQ ID NO: 34 - protein, 248 aa, Artificial sequence
  Anti-P329G-scFv
EVKLLESGGGLVQPGGSLKLSCAASGFDFSRYWMNWVRQAPGKGLEWIGEITPDSSTINYTPSLKDKFIISRDNAKNTLYLQMIKVRSEDTALYYCVRPYDYGAWFASWGQGTLVTVSAGGGGSGGGGSGGGGSGGGGSQAVVTQESALTTSPGETVTLTCRSSTGAVTTSNYANWVQEKPDHLFTGLIGGTNKRAPGVPARFSGSLIGDKAALTITGAQTEDEAIYFCALWYSNHWVFGGGTKLTVL

SEQ ID NO: 35 - DNA, 1356 bp, Artificial sequence
  Anti-P329G-scFv-CD28ATM-CD28CSD-CD3zSSD fusion
atgggatggagctgtatcatcctcttcttggtagcaacagctaccggtgtgcattccgaggtgaagctgctggagagcggcggcggcctggtgcagcccggcggcagcctgaagctgagctgcgccgccagcggcttcgacttcagcaggtactggatgaactgggtgaggcaggcccccggcaagggtctggagtggatcggcgagatcacccccgacagcagcaccatcaactacacccccagcctgaaggacaagttcatcatcagcagggacaacgccaagaacaccctgtacctgcagatgatcaaggtgaggagcgaggacaccgccctgtactactgcgtgaggccctacgactacggcgcctggttcgccagctggggccagggcaccctggtgaccgtgagcgccggagggggcggaagtggtggcgggggaagcggcgggggtggcagcggagggggcggatctcaggccgtggtgacccaggagagcgccctgaccaccagccccggcgagaccgtgaccctgacctgcaggagcagcaccggcgccgtgaccaccagcaactacgccaactgggtgcaggagaagcccgaccacctgttcaccggcctgatcggcggcaccaacaagagggcccccggcgtgcccgccaggttcagcggcagcctgatcggcgacaaggccgccctgaccatcaccggcgcccagaccgaggacgaggccatctacttctgcgccctgtggtacagcaaccactgggtgttcggcggtggcaccaagctgaccgtgctgggagggggcggatccttctgggtgctggtggtggtgggcggcgtgctggcctgctacagcctgctggtgaccgtggccttcatcatcttctgggtgaggagcaagaggagcaggctgctgcacagcgactacatgaacatgacccccaggaggcccggccccaccaggaagcactaccagccctacgccccccccagggacttcgccgcctacaggagcagggtgaagttcagcaggagcgccgacgcccccgcctaccagcagggccagaaccagctgtataacgagctgaacctgggcaggagggaggagtacgacgtgctggacaagaggaggggcagggaccccgagatgggcggcaagcccaggaggaagaacccccaggagggcctgtataacgagctgcagaaggacaagatggccgaggcctacagcgagatcggcatgaagggcgagaggaggaggggcaagggccacgacggcctgtaccagggcctgagcaccgccaccaaggacacctacgacgccctgcacatgcaggccctgccccccagg

SEQ ID NO: 36 - DNA, 357 bp, Artificial sequence
  Anti-P329G VH
gaggtgaagctgctggagagcggcggcggcctggtgcagcccggcggcagcctgaagctgagctgcgccgccagcggcttcgacttcagcaggtactggatgaactgggtgaggcaggcccccggcaagggtctggagtggatcggcgagatcacccccgacagcagcaccatcaactacacccccagcctgaaggacaagttcatcatcagcagggacaacgccaagaacaccctgtacctgcagatgatcaaggtgaggagcgaggacaccgccctgtactactgcgtgaggccctacgactacggcgcctggttcgccagctggggccagggcaccctggtgaccgtgagcgcc

SEQ ID NO: 37 - DNA, 327 bp, Artificial sequence
  Anti-P329G VL
caggccgtggtgacccaggagagcgccctgaccaccagccccggcgagaccgtgaccctgacctgcaggagcagcaccggcgccgtgaccaccagcaactacgccaactgggtgcaggagaagcccgaccacctgttcaccggcctgatcggcggcaccaacaagagggcccccggcgtgcccgccaggttcagcggcagcctgatcggcgacaaggccgccctgaccatcaccggcgcccagaccgaggacgaggccatctacttctgcgccctgtggtacagcaaccactgggtgttcggcggtggcaccaagctgaccgtgctg

SEQ ID NO: 38 - DNA, 2136 bp, Artificial sequence
  Anti-P329G-scFv-CD28ATM-CD28CSD-CD3zSSD-eGFP fusion
atgggatggagctgtatcatcctcttcttggtagcaacagctaccggtgtgcattccgaggtgaagctgctggagagcggcggcggcctggtgcagcccggcggcagcctgaagctgagctgcgccgccagcggcttcgacttcagcaggtactggatgaactgggtgaggcaggcccccggcaagggtctggagtggatcggcgagatcacccccgacagcagcaccatcaactacacccccagcctgaaggacaagttcatcatcagcagggacaacgccaagaacaccctgtacctgcagatgatcaaggtgaggagcgaggacaccgccctgtactactgcgtgaggccctacgactacggcgcctggttcgccagctggggccagggcaccctggtgaccgtgagcgccggagggggcggaagtggtggcgggggaagcggcgggggtggcagcggagggggcggatctcaggccgtggtgacccaggagagcgccctgaccaccagccccggcgagaccgtgaccctgacctgcaggagcagcaccggcgccgtgaccaccagcaactacgccaactgggtgcaggagaagcccgaccacctgttcaccggcctgatcggcggcaccaacaagagggcccccggcgtgcccgccaggttcagcggcagcctgatcggcgacaaggccgccctgaccatcaccggcgcccagaccgaggacgaggccatctacttctgcgccctgtggtacagcaaccactgggtgttcggcggtggcaccaagctgaccgtgctgggagggggcggatccttctgggtgctggtggtggtgggcggcgtgctggcctgctacagcctgctggtgaccgtggccttcatcatcttctgggtgaggagcaagaggagcaggctgctgcacagcgactacatgaacatgacccccaggaggcccggccccaccaggaagcactaccagccctacgccccccccagggacttcgccgcctacaggagcagggtgaagttcagcaggagcgccgacgcccccgcctaccagcagggccagaaccagctgtataacgagctgaacctgggcaggagggaggagtacgacgtgctggacaagaggaggggcagggaccccgagatgggcggcaagcccaggaggaagaacccccaggagggcctgtataacgagctgcagaaggacaagatggccgaggcctacagcgagatcggcatgaagggcgagaggaggaggggcaagggccacgacggcctgtaccagggcctgagcaccgccaccaaggacacctacgacgccctgcacatgcaggccctgccccccaggtccggagagggcagaggaagtcttctaacatgcggtgacgtggaggagaatcccggccctagggtgagcaagggcgaggagctgttcaccggggtggtgcccatcctggtcgagctggacggcgacgtaaacggccacaagttcagcgtgtccggcgagggcgagggcgatgccacctacggcaagctgaccctgaagttcatctgcaccaccggcaagctgcccgtgccctggcccaccctcgtgaccaccctgacctacggcgtgcagtgcttcagccgctaccccgaccacatgaagcagcacgacttcttcaagtccgccatgcccgaaggctacgtccaggagcgcaccatcttcttcaaggacgacggcaactacaagacccgcgccgaggtgaagttcgagggcgacaccctggtgaaccgcatcgagctgaagggcatcgacttcaaggaggacggcaacatcctggggcacaagctggagtacaactacaacagccacaacgtctatatcatggccgacaagcagaagaacggcatcaaggtgaacttcaagatccgccacaacatcgaggacggcagcgtgcagctcgccgaccactaccagcagaacacccccatcggcgacggccccgtgctgctgcccgacaaccactacctgagcacccagtccgccctgagcaaagaccccaacgagaagcgcgatcacatggtcctgctggagttcgtgaccgccgccgggatcactctcggcatggacgagctgtacaagtga

SEQ ID NO: 39 - protein, 407 aa, Artificial sequence
  Anti-P329G-ds-Fab- heavy chain-CD28ATM-CD28CSD-CD3zSSD fusion pETR17100
EVKLLESGGGLVQPGGSLKLSCAASGFDFSRYWMNWVRQAPGKCLEWIGEITPDSSTINYTPSLKDKFIISRDNAKNTLYLQMIKVRSEDTALYYCVRPYDYGAWFASWGQGTLVTVSAASTKGPSVFPLAPSSKSTSGGTAALGCLVKDYFPEPVTVSWNSGALTSGVHTFPAVLQSSGLYSLSSVVTVPSSSLGTQTYICNVNHKPSNTKVDKKVEPKSCGGGGSFWVLVVVGGVLACYSLLVTVAFIIFWVRSKRSRLLHSDYMNMTPRRPGPTRKHYQPYAPPRDFAAYRSRVKFSRSADAPAYQQGQNQLYNELNLGRREEYDVLDKRRGRDPEMGGKPRRKNPQEGLYNELQKDKMAEAYSEIGMKGERRRGKGHDGLYQGLSTATKDTYDALHMQALPPR

SEQ ID NO: 40 - protein, 222 aa, Artificial sequence
  Anti-P329G-ds-Fab heavy chain
EVKLLESGGGLVQPGGSLKLSCAASGFDFSRYWMNWVRQAPGKCLEWIGEITPDSSTINYTPSLKDKFIISRDNAKNTLYLQMIKVRSEDTALYYCVRPYDYGAWFASWGQGTLVTVSAASTKGPSVFPLAPSSKSTSGGTAALGCLVKDYFPEPVTVSWNSGALTSGVHTFPAVLQSSGLYSLSSVVTVPSSSLGTQTYICNVNHKPSNTKVDKKVEPKSC

SEQ ID NO: 41 - protein, 216 aa, Artificial sequence
  Anti P329G-ds-Fab light chain
QAVVTQESALTTSPGETVTLTCRSSTGAVTTSNYANWVQEKPDHLFTGLIGGTNKRAPGVPARFSGSLIGDKAALTITGAQTEDEAIYFCALWYSNHWVFGCGTKLTVLRTVAAPSVFIFPPSDEQLKSGTASVVCLLNNFYPREAKVQWKVDNALQSGNSQESVTEQDSKDSTYSLSSTLTLSKADYEKHKVYACEVTHQGLSSPVTKSFNRGEC

SEQ ID NO: 42 - protein, 107 aa, Artificial sequence [sequence omitted]

SEQ ID NO: 43 - protein, 103 aa, Artificial sequence
  CH1
ASTKGPSVFPLAPSSKSTSGGTAALGCLVKDYFPEPVTVSWNSGALTSGVHTFPAVLQSSGLYSLSSVVTVPSSSLGTQTYICNVNHKPSNTKVDKKVEPKSC

SEQ ID NO: 44 - DNA, 2645 bp, Artificial sequence
  Anti-P329G-ds-Fab-heavy chain-CD28ATM-CD28CSD-CD3zSSD fusion pETR17100
atgggatggagctgtatcatcctcttcttggtagcaacagctacgggtgtgcattcccaggccgtggtgacccaggagagcgccctgaccaccagccccggcgagaccgtgaccctgacctgcaggagcagcaccggcgccgtgaccaccagcaactacgccaactgggtgcaggagaagcccgaccacctgttcaccggcctgatcggcggcaccaacaagagggcccccggcgtgcccgccaggttcagcggcagcctgatcggcgacaaggccgccctgaccatcaccggcgcccagaccgaggacgaggccatctacttctgcgccctgtggtacagcaaccactgggtgttcggctgtggcaccaagctgaccgtgctgcgtacggtggctgcaccatctgtcttcatcttcccgccatctgatgagcagttgaaatctggaactgcctctgttgtgtgcctgctgaataacttctatcccagagaggccaaagtacagtggaaggtggataacgccctccaatcgggtaactcccaggagagtgtcacagagcaggacagcaaggacagcacctacagcctcagcagcaccctgacgctgagcaaagcagactacgagaaacacaaagtctacgcctgcgaagtcacccatcagggcctgagctcgcccgtcacaaagagcttcaacaggggagagtgttaggaattccccgaagtaacttagaagctgtaaatcaacgatcaatagcaggtgtggcacaccagtcataccttgatcaagcacttctgtttccccggactgagtatcaataggctgctcgcgcggctgaaggagaaaacgttcgttacccgaccaactacttcgagaagcttagtaccaccatgaacgaggcagggtgtttcgctcagcacaaccccagtgtagatcaggctgatgagtcactgcaacccccatgggcgaccatggcagtggctgcgttggcggcctgcccatggagaaatccatgggacgctctaattctgacatggtgtgaagtgcctattgagctaactggtagtcctccggcccctgattgcggctaatcctaactgcggagcacatgctcacaaaccagtgggtggtgtgtcgtaacgggcaactctgcagcggaaccgactactttgggtgtccgtgtttccttttattcctatattggctgcttatggtgacaatcaaaaagttgttaccatatagctattggattggccatccggtgtgcaacagggcaactgtttacctatttattggttttgtaccattatcactgaagtctgtgatcactctcaaattcattttgaccctcaacacaatcaaacgccaccatgggatggagctgtatcatcctcttcttggtagcaacagctaccggtgtgcactccgaggtgaagctgctggagagcggcggcggcctggtgcagcccggcggcagcctgaagctgagctgcgccgccagcggcttcgacttcagcaggtactggatgaactgggtgaggcaggcccccggcaagtgtctggagtggatcggcgagatcacccccgacagcagcaccatcaactacacccccagcctgaaggacaagttcatcatcagcagggacaacgccaagaacaccctgtacctgcagatgatcaaggtgaggagcgaggacaccgccctgtactactgcgtgaggccctacgactacggcgcctggttcgccagctggggccagggcaccctggtgaccgtgagcgccgctagcaccaagggcccctccgtgttccccctggcccccagcagcaagagcaccagcggcggcacagccgctctgggctgcctggtcaaggactacttccccgagcccgtgaccgtgtcctggaacagcggagccctgacctccggcgtgcacaccttccccgccgtgctgcagagttctggcctgtatagcctgagcagcgtggtcaccgtgccttctagcagcctgggcacccagacctacatctgcaacgtgaaccacaagcccagcaacaccaaggtggacaagaaggtggagcccaagagctgcggagggggcggatccttctgggtgctggtggtggtgggcggcgtgctggcctgctacagcctgctggtgaccgtggccttcatcatcttctgggtgaggagcaagaggagcaggctgctgcacagcgactacatgaacatgacccccaggaggcccggccccaccaggaagcactaccagccctacgccccccccagggacttcgccgcctacaggagcagggtgaagttcagcaggagcgccgacgcccccgcctaccagcagggccagaaccagctgtataacgagctgaacctgggcaggagggaggagtacgacgtgctggacaagaggaggggcagggaccccgagatgggcggcaagcccaggaggaagaacccccaggagggcctgtataacgagctgcagaaggacaagatggccgaggcctacagcgagatcggcatgaagggcgagaggaggaggggcaagggccacgacggcctgtaccagggcctgagcaccgccaccaaggacacctacgacgccctgcacatgcaggccctgccccccagg

SEQ ID NO: 45 - DNA, 324 bp, Artificial sequence
  CL
cgtacggtggctgcaccatctgtcttcatcttcccgccatctgatgagcagttgaaatctggaactgcctctgttgtgtgcctgctgaataacttctatcccagagaggccaaagtacagtggaaggtggataacgccctccaatcgggtaactcccaggagagtgtcacagagcaggacagcaaggacagcacctacagcctcagcagcaccctgacgctgagcaaagcagactacgagaaacacaaagtctacgcctgcgaagtcacccatcagggcctgagctcgcccgtcacaaagagcttcaacaggggagagtgttag

SEQ ID NO: 46 - DNA, 309 bp, Artificial sequence
  CH1
gctagcaccaagggcccctccgtgttccccctggcccccagcagcaagagcaccagcggcggcacagccgctctgggctgcctggtcaaggactacttccccgagcccgtgaccgtgtcctggaacagcggagccctgacctccggcgtgcacaccttccccgccgtgctgcagagttctggcctgtatagcctgagcagcgtggtcaccgtgccttctagcagcctgggcacccagacctacatctgcaacgtgaaccacaagcccagcaacaccaaggtggacaagaaggtggagcccaagagctgc

SEQ ID NO: 47 - DNA, 3425 bp, Artificial sequence
  Anti-P329G-ds-Fab-heavy chain-CD28TM-CD28CSD-CD3ZSSD-eGFP fusion pETR17100
atgggatggagctgtatcatcctcttcttggtagcaacagctacgggtgtgcattcccaggccgtggtgacccaggagagcgccctgaccaccagccccggcgagaccgtgaccctgacctgcaggagcagcaccggcgccgtgaccaccagcaactacgccaactgggtgcaggagaagcccgaccacctgttcaccggcctgatcggcggcaccaacaagagggcccccggcgtgcccgccaggttcagcggcagcctgatcggcgacaaggccgccctgaccatcaccggcgcccagaccgaggacgaggccatctacttctgcgccctgtggtacagcaaccactgggtgttcggctgtggcaccaagctgaccgtgctgcgtacggtggctgcaccatctgtcttcatcttcccgccatctgatgagcagttgaaatctggaactgcctctgttgtgtgcctgctgaataacttctatcccagagaggccaaagtacagtggaaggtggataacgccctccaatcgggtaactcccaggagagtgtcacagagcaggacagcaaggacagcacctacagcctcagcagcaccctgacgctgagcaaagcagactacgagaaacacaaagtctacgcctgcgaagtcacccatcagggcctgagctcgcccgtcacaaagagcttcaacaggggagagtgttaggaattccccgaagtaacttagaagctgtaaatcaacgatcaatagcaggtgtggcacaccagtcataccttgatcaagcacttctgtttccccggactgagtatcaataggctgctcgcgcggctgaaggagaaaacgttcgttacccgaccaactacttcgagaagcttagtaccaccatgaacgaggcagggtgtttcgctcagcacaaccccagtgtagatcaggctgatgagtcactgcaacccccatgggcgaccatggcagtggctgcgttggcggcctgcccatggagaaatccatgggacgctctaattctgacatggtgtgaagtgcctattgagctaactggtagtcctccggcccctgattgcggctaatcctaactgcggagcacatgctcacaaaccagtgggtggtgtgtcgtaacgggcaactctgcagcggaaccgactactttgggtgtccgtgtttccttttattcctatattggctgcttatggtgacaatcaaaaagttgttaccatatagctattggattggccatccggtgtgcaacagggcaactgtttacctatttattggttttgtaccattatcactgaagtctgtgatcactctcaaattcattttgaccctcaacacaatcaaacgccaccatgggatggagctgtatcatcctcttcttggtagcaacagctaccggtgtgcactccgaggtgaagctgctggagagcggcggcggcctggtgcagcccggcggcagcctgaagctgagctgcgccgccagcggcttcgacttcagcaggtactggatgaactgggtgaggcaggcccccggcaagtgtctggagtggatcggcgagatcacccccgacagcagcaccatcaactacacccccagcctgaaggacaagttcatcatcagcagggacaacgccaagaacaccctgtacctgcagatgatcaaggtgaggagcgaggacaccgccctgtactactgcgtgaggccctacgactacggcgcctggttcgccagctggggccagggcaccctggtgaccgtgagcgccgctagcaccaagggcccctccgtgttccccctggcccccagcagcaagagcaccagcggcggcacagccgctctgggctgcctggtcaaggactacttccccgagcccgtgaccgtgtcctggaacagcggagccctgacctccggcgtgcacaccttccccgccgtgctgcagagttctggcctgtatagcctgagcagcgtggtcaccgtgccttctagcagcctgggcacccagacctacatctgcaacgtgaaccacaagcccagcaacaccaaggtggacaagaaggtggagcccaagagctgcggagggggcggatccttctgggtgctggtggtggtgggcggcgtgctggcctgctacagcctgctggtgaccgtggccttcatcatcttctgggtgaggagcaagaggagcaggctgctgcacagcgactacatgaacatgacccccaggaggcccggccccaccaggaagcactaccagccctacgccccccccagggacttcgccgcctacaggagcagggtgaagttcagcaggagcgccgacgcccccgcctaccagcagggccagaaccagctgtataacgagctgaacctgggcaggagggaggagtacgacgtgctggacaagaggaggggcagggaccccgagatgggcggcaagcccaggaggaagaacccccaggagggcctgtataacgagctgcagaaggacaagatggccgaggcctacagcgagatcggcatgaagggcgagaggaggaggggcaagggccacgacggcctgtaccagggcctgagcaccgccaccaaggacacctacgacgccctgcacatgcaggccctgccccccaggtccggagagggcagaggaagtcttctaacatgcggtgacgtggaggagaatcccggccctagggtgagcaagggcgaggagctgttcaccggggtggtgcccatcctggtcgagctggacggcgacgtaaacggccacaagttcagcgtgtccggcgagggcgagggcgatgccacctacggcaagctgaccctgaagttcatctgcaccaccggcaagctgcccgtgccctggcccaccctcgtgaccaccctgacctacggcgtgcagtgcttcagccgctaccccgaccacatgaagcagcacgacttcttcaagtccgccatgcccgaaggctacgtccaggagcgcaccatcttcttcaaggacgacggcaactacaagacccgcgccgaggtgaagttcgagggcgacaccctggtgaaccgcatcgagctgaagggcatcgacttcaaggaggacggcaacatcctggggcacaagctggagtacaactacaacagccacaacgtctatatcatggccgacaagcagaagaacggcatcaaggtgaacttcaagatccgccacaacatcgaggacggcagcgtgcagctcgccgaccactaccagcagaacacccccatcggcgacggccccgtgctgctgcccgacaaccactacctgagcacccagtccgccctgagcaaagaccccaacgagaagcgcgatcacatggtcctgctggagttcgtgaccgccgccgggatcactctcggcatggacgagctgtacaagtga

SEQ ID NO: 48 - protein, 407 aa, Artificial sequence
  Anti-P329G-Fab-heavy chain-CD28ATM-CD28CSD-CD3zSSD fusion pETR17594
EVKLLESGGGLVQPGGSLKLSCAASGFDFSRYWMNWVRQAPGKGLEWIGEITPDSSTINYTPSLKDKFIISRDNAKNTLYLQMIKVRSEDTALYYCVRPYDYGAWFASWGQGTLVTVSAASTKGPSVFPLAPSSKSTSGGTAALGCLVKDYFPEPVTVSWNSGALTSGVHTFPAVLQSSGLYSLSSVVTVPSSSLGTQTYICNVNHKPSNTKVDKKVEPKSCGGGGSFWVLVVVGGVLACYSLLVTVAFIIFWVRSKRSRLLHSDYMNMTPRRPGPTRKHYQPYAPPRDFAAYRSRVKFSRSADAPAYQQGQNQLYNELNLGRREEYDVLDKRRGRDPEMGGKPRRKNPQEGLYNELQKDKMAEAYSEIGMKGERRRGKGHDGLYQGLSTATKDTYDALHMQALPPR

SEQ ID NO: 49 - protein, 222 aa, Artificial sequence
  Anti-P329G-Fab heavy chain
EVKLLESGGGLVQPGGSLKLSCAASGFDFSRYWMNWVRQAPGKGLEWIGEITPDSSTINYTPSLKDKFIISRDNAKNTLYLQMIKVRSEDTALYYCVRPYDYGAWFASWGQGTLVTVSAASTKGPSVFPLAPSSKSTSGGTAALGCLVKDYFPEPVTVSWNSGALTSGVHTFPAVLQSSGLYSLSSVVTVPSSSLGTQTYICNVNHKPSNTKVDKKVEPKSC

SEQ ID NO: 50 - protein, 216 aa, Artificial sequence
  Anti-P329G-Fab light chain
QAVVTQESALTTSPGETVTLTCRSSTGAVTTSNYANWVQEKPDHLFTGLIGGTNKRAPGVPARFSGSLIGDKAALTITGAQTEDEAIYFCALWYSNHWVFGGGTKLTVLRTVAAPSVFIFPPSDEQLKSGTASVVCLLNNFYPREAKVQWKVDNALQSGNSQESVTEQDSKDSTYSLSSTLTLSKADYEKHKVYACEVTHQGLSSPVTKSFNRGEC

SEQ ID NO: 51 - DNA, 2645 bp, Artificial sequence
  Anti-P329G-Fab-heavy chain-CD28ATM-CD28CSD-CD3zSSD fusion pETR17594
atgggatggagctgtatcatcctcttcttggtagcaacagctacgggtgtgcattcccaggccgtggtgacccaggagagcgccctgaccaccagccccggcgagaccgtgaccctgacctgcaggagcagcaccggcgccgtgaccaccagcaactacgccaactgggtgcaggagaagcccgaccacctgttcaccggcctgatcggcggcaccaacaagagggcccccggcgtgcccgccaggttcagcggcagcctgatcggcgacaaggccgccctgaccatcaccggcgcccagaccgaggacgaggccatctacttctgcgccctgtggtacagcaaccactgggtgttcggcggtggcaccaagctgaccgtgctgcgtacggtggctgcaccatctgtcttcatcttcccgccatctgatgagcagttgaaatctggaactgcctctgttgtgtgcctgctgaataacttctatcccagagaggccaaagtacagtggaaggtggataacgccctccaatcgggtaactcccaggagagtgtcacagagcaggacagcaaggacagcacctacagcctcagcagcaccctgacgctgagcaaagcagactacgagaaacacaaagtctacgcctgcgaagtcacccatcagggcctgagctcgcccgtcacaaagagcttcaacaggggagagtgttaggaattccccgaagtaacttagaagctgtaaatcaacgatcaatagcaggtgtggcacaccagtcataccttgatcaagcacttctgtttccccggactgagtatcaataggctgctcgcgcggctgaaggagaaaacgttcgttacccgaccaactacttcgagaagcttagtaccaccatgaacgaggcagggtgtttcgctcagcacaaccccagtgtagatcaggctgatgagtcactgcaacccccatgggcgaccatggcagtggctgcgttggcggcctgcccatggagaaatccatgggacgctctaattctgacatggtgtgaagtgcctattgagctaactggtagtcctccggcccctgattgcggctaatcctaactgcggagcacatgctcacaaaccagtgggtggtgtgtcgtaacgggcaactctgcagcggaaccgactactttgggtgtccgtgtttccttttattcctatattggctgcttatggtgacaatcaaaaagttgttaccatatagctattggattggccatccggtgtgcaacagggcaactgtttacctatttattggttttgtaccattatcactgaagtctgtgatcactctcaaattcattttgaccctcaacacaatcaaacgccaccatgggatggagctgtatcatcctcttcttggtagcaacagctaccggtgtgcactccgaggtgaagctgctggagagcggcggcggcctggtgcagcccggcggcagcctgaagctgagctgcgccgccagcggcttcgacttcagcaggtactggatgaactgggtgaggcaggcccccggcaagggtctggagtggatcggcgagatcacccccgacagcagcaccatcaactacacccccagcctgaaggacaagttcatcatcagcagggacaacgccaagaacaccctgtacctgcagatgatcaaggtgaggagcgaggacaccgccctgtactactgcgtgaggccctacgactacggcgcctggttcgccagctggggccagggcaccctggtgaccgtgagcgccgctagcaccaagggcccctccgtgttccccctggcccccagcagcaagagcaccagcggcggcacagccgctctgggctgcctggtcaaggactacttccccgagcccgtgaccgtgtcctggaacagcggagccctgacctccggcgtgcacaccttccccgccgtgctgcagagttctggcctgtatagcctgagcagcgtggtcaccgtgccttctagcagcctgggcacccagacctacatctgcaacgtgaaccacaagcccagcaacaccaaggtggacaagaaggtggagcccaagagctgcggagggggcggatccttctgggtgctggtggtggtgggcggcgtgctggcctgctacagcctgctggtgaccgtggccttcatcatcttctgggtgaggagcaagaggagcaggctgctgcacagcgactacatgaacatgacccccaggaggcccggccccaccaggaagcactaccagccctacgccccccccagggacttcgccgcctacaggagcagggtgaagttcagcaggagcgccgacgcccccgcctaccagcagggccagaaccagctgtataacgagctgaacctgggcaggagggaggagtacgacgtgctggacaagaggaggggcagggaccccgagatgggcggcaagcccaggaggaagaacccccaggagggcctgtataacgagctgcagaaggacaagatggccgaggcctacagcgagatcggcatgaagggcgagaggaggaggggcaagggccacgacggcctgtaccagggcctgagcaccgccaccaaggacacctacgacgccctgcacatgcaggccctgccccccagg

SEQ ID NO: 52 - DNA, 3425 bp, Artificial sequence
  Anti-P329G-Fab-heavy chain-CD28ATM-CD28CSD-CD3zSSD-eGFP fusion pETR17594
atgggatggagctgtatcatcctcttcttggtagcaacagctacgggtgtgcattcccaggccgtggtgacccaggagagcgccctgaccaccagccccggcgagaccgtgaccctgacctgcaggagcagcaccggcgccgtgaccaccagcaactacgccaactgggtgcaggagaagcccgaccacctgttcaccggcctgatcggcggcaccaacaagagggcccccggcgtgcccgccaggttcagcggcagcctgatcggcgacaaggccgccctgaccatcaccggcgcccagaccgaggacgaggccatctacttctgcgccctgtggtacagcaaccactgggtgttcggcggtggcaccaagctgaccgtgctgcgtacggtggctgcaccatctgtcttcatcttcccgccatctgatgagcagttgaaatctggaactgcctctgttgtgtgcctgctgaataacttctatcccagagaggccaaagtacagtggaaggtggataacgccctccaatcgggtaactcccaggagagtgtcacagagcaggacagcaaggacagcacctacagcctcagcagcaccctgacgctgagcaaagcagactacgagaaacacaaagtctacgcctgcgaagtcacccatcagggcctgagctcgcccgtcacaaagagcttcaacaggggagagtgttaggaattccccgaagtaacttagaagctgtaaatcaacgatcaatagcaggtgtggcacaccagtcataccttgatcaagcacttctgtttccccggactgagtatcaataggctgctcgcgcggctgaaggagaaaacgttcgttacccgaccaactacttcgagaagcttagtaccaccatgaacgaggcagggtgtttcgctcagcacaaccccagtgtagatcaggctgatgagtcactgcaacccccatgggcgaccatggcagtggctgcgttggcggcctgcccatggagaaatccatgggacgctctaattctgacatggtgtgaagtgcctattgagctaactggtagtcctccggcccctgattgcggctaatcctaactgcggagcacatgctcacaaaccagtgggtggtgtgtcgtaacgggcaactctgcagcggaaccgactactttgggtgtccgtgtttccttttattcctatattggctgcttatggtgacaatcaaaaagttgttaccatatagctattggattggccatccggtgtgcaacagggcaactgtttacctatttattggttttgtaccattatcactgaagtctgtgatcactctcaaattcattttgaccctcaacacaatcaaacgccaccatgggatggagctgtatcatcctcttcttggtagcaacagctaccggtgtgcactccgaggtgaagctgctggagagcggcggcggcctggtgcagcccggcggcagcctgaagctgagctgcgccgccagcggcttcgacttcagcaggtactggatgaactgggtgaggcaggcccccggcaagggtctggagtggatcggcgagatcacccccgacagcagcaccatcaactacacccccagcctgaaggacaagttcatcatcagcagggacaacgccaagaacaccctgtacctgcagatgatcaaggtgaggagcgaggacaccgccctgtactactgcgtgaggccctacgactacggcgcctggttcgccagctggggccagggcaccctggtgaccgtgagcgccgctagcaccaagggcccctccgtgttccccctggcccccagcagcaagagcaccagcggcggcacagccgctctgggctgcctggtcaaggactacttccccgagcccgtgaccgtgtcctggaacagcggagccctgacctccggcgtgcacaccttccccgccgtgctgcagagttctggcctgtatagcctgagcagcgtggtcaccgtgccttctagcagcctgggcacccagacctacatctgcaacgtgaaccacaagcccagcaacaccaaggtggacaagaaggtggagcccaagagctgcggagggggcggatccttctgggtgctggtggtggtgggcggcgtgctggcctgctacagcctgctggtgaccgtggccttcatcatcttctgggtgaggagcaagaggagcaggctgctgcacagcgactacatgaacatgacccccaggaggcccggccccaccaggaagcactaccagccctacgccccccccagggacttcgccgcctacaggagcagggtgaagttcagcaggagcgccgacgcccccgcctaccagcagggccagaaccagctgtataacgagctgaacctgggcaggagggaggagtacgacgtgctggacaagaggaggggcagggaccccgagatgggcggcaagcccaggaggaagaacccccaggagggcctgtataacgagctgcagaaggacaagatggccgaggcctacagcgagatcggcatgaagggcgagaggaggaggggcaagggccacgacggcctgtaccagggcctgagcaccgccaccaaggacacctacgacgccctgcacatgcaggccctgccccccaggtccggagagggcagaggaagtcttctaacatgcggtgacgtggaggagaatcccggccctagggtgagcaagggcgaggagctgttcaccggggtggtgcccatcctggtcgagctggacggcgacgtaaacggccacaagttcagcgtgtccggcgagggcgagggcgatgccacctacggcaagctgaccctgaagttcatctgcaccaccggcaagctgcccgtgccctggcccaccctcgtgaccaccctgacctacggcgtgcagtgcttcagccgctaccccgaccacatgaagcagcacgacttcttcaagtccgccatgcccgaaggctacgtccaggagcgcaccatcttcttcaaggacgacggcaactacaagacccgcgccgaggtgaagttcgagggcgacaccctggtgaaccgcatcgagctgaagggcatcgacttcaaggaggacggcaacatcctggggcacaagctggagtacaactacaacagccacaacgtctatatcatggccgacaagcagaagaacggcatcaaggtgaacttcaagatccgccacaacatcgaggacggcagcgtgcagctcgccgaccactaccagcagaacacccccatcggcgacggccccgtgctgctgcccgacaaccactacctgagcacccagtccgccctgagcaaagaccccaacgagaagcgcgatcacatggtcctgctggagttcgtgaccgccgccgggatcactctcggcatggacgagctgtacaagtga

SEQ ID NO: 53 - protein, 5 aa, Artificial sequence
  Anti-AAA CDR H1 Kabat
SYGMS

SEQ ID NO: 54 - protein, 6 aa, Artificial sequence
  Anti-AAA CDR H2 Kabat
SSGGSY

SEQ ID NO: 55 - protein, 12 aa, Artificial sequence
  Anti-AAA CDR H3 Kabat
LGMITTGYAMDY

SEQ ID NO: 56 - protein, 16 aa, Artificial sequence
  Anti-AAA CDR L1 Kabat
RSSQTIVHSTGHTYLE

SEQ ID NO: 57 - protein, 7 aa, Artificial sequence
  Anti-AAA CDR L2 Kabat
KVSNRFS

SEQ ID NO: 58 - protein, 9 aa, Artificial sequence
  Anti-AAA CDR L3 Kabat
FQGSHVPYT

SEQ ID NO: 59 - protein, 457 aa, Artificial sequence
  Anti-AAA-scFv-CD28ATM-CD28CSD-CD3zSSD fusion
MNFGLSLVFLALILKGVQCEVQLVESGGDLVKPGGSLKLSCAASGFTFSSYGMSWVRQTPDKRLEWVATISSGGSYIYYPDSVKGRFTISRDNAKNTLYLQMSSLKSEDTAMYYCARLGMITTGYAMDYWGQGTSVTVSSGGGGSGGGGSGGGGSGGGGSDVLMTQTPLSLPVSLGDQASISCRSSQTIVHSTGHTYLEWFLQKPGQSPKLLIYKVSNRFSGVPDRFSGSGSGTDFTLKISRVEAEDLGVYYCFQGSHVPYTFGGGTKLEIKGGGGSFWVLVVVGGVLACYSLLVTVAFIIFWVRSKRSRLLHSDYMNMTPRRPGPTRKHYQPYAPPRDFAAYRSRVKFSRSADAPAYQQGQNQLYNELNLGRREEYDVLDKRRGRDPEMGGKPRRKNPQEGLYNELQKDKMAEAYSEIGMKGERRRGKGHDGLYQGLSTATKDTYDALHMQALPPR

SEQ ID NO: 60 - protein, 272 aa, Artificial sequence
  Anti-AAA-scFv
MNFGLSLVFLALILKGVQCEVQLVESGGDLVKPGGSLKLSCAASGFTFSSYGMSWVRQTPDKRLEWVATISSGGSYIYYPDSVKGRFTISRDNAKNTLYLQMSSLKSEDTAMYYCARLGMITTGYAMDYWGQGTSVTVSSGGGGSGGGGSGGGGSGGGGSDVLMTQTPLSLPVSLGDQASISCRSSQTIVHSTGHTYLEWFLQKPGQSPKLLIYKVSNRFSGVPDRFSGSGSGTDFTLKISRVEAEDLGVYYCFQGSHVPYTFGGGTKLEIK

SEQ ID NO: 61 - protein, 140 aa, Artificial sequence
  Anti-AAA VH
MNFGLSLVFLALILKGVQCEVQLVESGGDLVKPGGSLKLSCAASGFTFSSYGMSWVRQTPDKRLEWVATISSGGSYIYYPDSVKGRFTISRDNAKNTLYLQMSSLKSEDTAMYYCARLGMITTGYAMDYWGQGTSVTVSS

SEQ ID NO: 62 - protein, 112 aa, Artificial sequence
  Anti-AAA VL
DVLMTQTPLSLPVSLGDQASISCRSSQTIVHSTGHTYLEWFLQKPGQSPKLLIYKVSNRFSGVPDRFSGSGSGTDFTLKISRVEAEDLGVYYCFQGSHVPYTFGGGTKLEIK

SEQ ID NO: 63 - protein, 428 aa, Artificial sequence
  Anti-AAA-Fab-heavy chain-CD28ATM-CD28CSD-CD3zSSD fusion
MNFGLSLVFLALILKGVQCEVQLVESGGDLVKPGGSLKLSCAASGFTFSSYGMSWVRQTPDKRLEWVATISSGGSYIYYPDSVKGRFTISRDNAKNTLYLQMSSLKSEDTAMYYCARLGMITTGYAMDYWGQGTSVTVSSASTKGPSVFPLAPSSKSTSGGTAALGCLVKDYFPEPVTVSWNSGALTSGVHTFPAVLQSSGLYSLSSVVTVPSSSLGTQTYICNVNHKPSNTKVDKKVEPKSCGGGGSFWVLVVVGGVLACYSLLVTVAFIIFWVRSKRSRLLHSDYMNMTPRRPGPTRKHYQPYAPPRDFAAYRSRVKFSRSADAPAYQQGQNQLYNELNLGRREEYDVLDKRRGRDPEMGGKPRRKNPQEGLYNELQKDKMAEAYSEIGMKGERRRGKGHDGLYQGLSTATKDTYDALHMQALPPR

SEQ ID NO: 64 - protein, 243 aa, Artificial sequence
  Anti-AAA-Fab heavy chain
MNFGLSLVFLALILKGVQCEVQLVESGGDLVKPGGSLKLSCAASGFTFSSYGMSWVRQTPDKRLEWVATISSGGSYIYYPDSVKGRFTISRDNAKNTLYLQMSSLKSEDTAMYYCARLGMITTGYAMDYWGQGTSVTVSSASTKGPSVFPLAPSSKSTSGGTAALGCLVKDYFPEPVTVSWNSGALTSGVHTFPAVLQSSGLYSLSSVVTVPSSSLGTQTYICNVNHKPSNTKVDKKVEPKSC

SEQ ID NO: 65 - protein, 219 aa, Artificial sequence
  Anti-AAA-Fab light chain
DVLMTQTPLSLPVSLGDQASISCRSSQTIVHSTGHTYLEWFLQKPGQSPKLLIYKVSNRFSGVPDRFSGSGSGTDFTLKISRVEAEDLGVYYCFQGSHVPYTFGGGTKLEIKRTVAAPSVFIFPPSDEQLKSGTASVVCLLNNFYPREAKVQWKVDNALQSGNSQESVTEQDSKDSTYSLSSTLTLSKADYEKHKVYACEVTHQGLSSPVTKSFNRGEC

SEQ ID NO: 66 - DNA, 780 bp, Homo sapiens
atggcgcgcccgcatccgtggtggctgtgcgtgctgggcaccctggtgggcctgagcgcgaccccggcgccgaaaagctgcccggaacgccattattgggcgcagggcaaactgtgctgccagatgtgcgaaccgggcacctttctggtgaaagattgcgatcagcatcgcaaagcggcgcagtgcgatccgtgcattccgggcgtgagctttagcccggatcatcatacccgcccgcattgcgaaagctgccgccattgcaacagcggcctgctggtgcgcaactgcaccattaccgcgaacgcggaatgcgcgtgccgcaacggctggcagtgccgcgataaagaatgcaccgaatgcgatccgctgccgaacccgagcctgaccgcgcgcagcagccaggcgctgagcccgcatccgcagccgacccatctgccgtatgtgagcgaaatgctggaagcgcgcaccgcgggccatatgcagaccctggcggattttcgccagctgccggcgcgcaccctgagcacccattggccgccgcagcgcagcctgtgcagcagcgattttattcgcattctggtgatttttagcggcatgtttctggtgtttaccctggcgggcgcgctgtttctgcatcagcgccgcaaatatcgcagcaacaaaggcgaaagcccggtggaaccggcggaaccgtgccattatagctgcccgcgcgaagaagaaggcagcaccattccgattcaggaagattatcgcaaaccggaaccggcgtgcagcccg

SEQ ID NO: 67 - protein, 260 aa, Homo sapiens
MARPHPWWLCVLGTLVGLSATPAPKSCPERHYWAQGKLCCQMCEPGTFLVKDCDQHRKAAQCDPCIPGVSFSPDHHTRPHCESCRHCNSGLLVRNCTITANAECACRNGWQCRDKECTECDPLPNPSLTARSSQALSPHPQPTHLPYVSEMLEARTAGHMQTLADFRQLPARTLSTHWPPQRSLCSSDFIRILVIFSGMFLVFTLAGALFLHQRRKYRSNKGESPVEPAEPCHYSCPREEEGSTIPIQEDYRKPEPACSP

SEQ ID NO: 68 - DNA, 750 bp, Mus musculus
atggcgtggccgccgccgtattggctgtgcatgctgggcaccctggtgggcctgagcgcgaccctggcgccgaacagctgcccggataaacattattggaccggcggcggcctgtgctgccgcatgtgcgaaccgggcaccttttttgtgaaagattgcgaacaggatcgcaccgcggcgcagtgcgatccgtgcattccgggcaccagctttagcccggattatcatacccgcccgcattgcgaaagctgccgccattgcaacagcggctttctgattcgcaactgcaccgtgaccgcgaacgcggaatgcagctgcagcaaaaactggcagtgccgcgatcaggaatgcaccgaatgcgatccgccgctgaacccggcgctgacccgccagccgagcgaaaccccgagcccgcagccgccgccgacccatctgccgcatggcaccgaaaaaccgagctggccgctgcatcgccagctgccgaacagcaccgtgtatagccagcgcagcagccatcgcccgctgtgcagcagcgattgcattcgcatttttgtgacctttagcagcatgtttctgatttttgtgctgggcgcgattctgttttttcatcagcgccgcaaccatggcccgaacgaagatcgccaggcggtgccggaagaaccgtgcccgtatagctgcccgcgcgaagaagaaggcagcgcgattccgattcaggaagattatcgcaaaccggaaccggcgttttatccg

SEQ ID NO: 69 - protein, 250 aa, Mus musculus
MAWPPPYWLCMLGTLVGLSATLAPNSCPDKHYWTGGGLCCRMCEPGTFFVKDCEQDRTAAQCDPCIPGTSFSPDYHTRPHCESCRHCNSGFLIRNCTVTANAECSCSKNWQCRDQECTECDPPLNPALTRQPSETPSPQPPPTHLPHGTEKPSWPLHRQLPNSTVYSQRSSHRPLCSSDCIRIFVTFSSMFLIFVLGAILFFHQRRNHGPNEDRQAVPEEPCPYSCPREEEGSAIPIQEDYRKPEPAFYP

SEQ ID NO: 70 - DNA, 660 bp, Homo sapiens
atgctgcgcctgctgctggcgctgaacctgtttccgagcattcaggtgaccggcaacaaaattctggtgaaacagagcccgatgctggtggcgtatgataacgcggtgaacctgagctgcaaatatagctataacctgtttagccgcgaatttcgcgcgagcctgcataaaggcctggatagcgcggtggaagtgtgcgtggtgtatggcaactatagccagcagctgcaggtgtatagcaaaaccggctttaactgcgatggcaaactgggcaacgaaagcgtgaccttttatctgcagaacctgtatgtgaaccagaccgatatttatttttgcaaaattgaagtgatgtatccgccgccgtatctggataacgaaaaaagcaacggcaccattattcatgtgaaaggcaaacatctgtgcccgagcccgctgtttccgggcccgagcaaaccgttttgggtgctggtggtggtgggcggcgtgctggcgtgctatagcctgctggtgaccgtggcgtttattattttttgggtgcgcagcaaacgcagccgcctgctgcatagcgattatatgaacatgaccccgcgccgcccgggcccgacccgcaaacattatcagccgtatgcgccgccgcgcgattttgcggcgtatcgcagc

SEQ ID NO: 71 - protein, 220 aa, Homo sapiens
MLRLLLALNLFPSIQVTGNKILVKQSPMLVAYDNAVNLSCKYSYNLFSREFRASLHKGLDSAVEVCVVYGNYSQQLQVYSKTGFNCDGKLGNESVTFYLQNLYVNQTDIYFCKIEVMYPPPYLDNEKSNGTIIHVKGKHLCPSPLFPGPSKPFWVLVVVGGVLACYSLLVTVAFIIFWVRSKRSRLLHSDYMNMTPRRPGPTRKHYQPYAPPRDFAAYRS

SEQ ID NO: 72 - DNA, 654 bp, Mus musculus
atgaccctgcgcctgctgtttctggcgctgaacttttttagcgtgcaggtgaccgaaaacaaaattctggtgaaacagagcccgctgctggtggtggatagcaacgaagtgagcctgagctgccgctatagctataacctgctggcgaaagaatttcgcgcgagcctgtataaaggcgtgaacagcgatgtggaagtgtgcgtgggcaacggcaactttacctatcagccgcagtttcgcagcaacgcggaatttaactgcgatggcgattttgataacgaaaccgtgacctttcgcctgtggaacctgcatgtgaaccataccgatatttatttttgcaaaattgaatttatgtatccgccgccgtatctggataacgaacgcagcaacggcaccattattcatattaaagaaaaacatctgtgccatacccagagcagcccgaaactgttttgggcgctggtggtggtggcgggcgtgctgttttgctatggcctgctggtgaccgtggcgctgtgcgtgatttggaccaacagccgccgcaaccgcctgctgcagagcgattatatgaacatgaccccgcgccgcccgggcctgacccgcaaaccgtatcagccgtatgcgccggcgcgcgattttgcggcgtatcgcccg

SEQ ID NO: 73 - protein, 218 aa, Mus musculus
MTLRLLFLALNFFSVQVTENKILVKQSPLLVVDSNEVSLSCRYSYNLLAKEFRASLYKGVNSDVEVCVGNGNFTYQPQFRSNAEFNCDGDFDNETVTFRLWNLHVNHTDIYFCKIEFMYPPPYLDNERSNGTIIHIKEKHLCHTQSSPKLFWALVVVAGVLFCYGLLVTVALCVIWTNSRRNRLLQSDYMNMTPRRPGLTRKPYQPYAPARDFAAYRP

SEQ ID NO: 74 - DNA, 768 bp, Homo sapiens
atgggaaacagctgttacaacatagtagccactctgttgctggtcctcaactttgagaggacaagatcattgcaggatccttgtagtaactgcccagctggtacattctgtgataataacaggaatcagatttgcagtccctgtcctccaaatagtttctccagcgcaggtggacaaaggacctgtgacatatgcaggcagtgtaaaggtgttttcaggaccaggaaggagtgttcctccaccagcaatgcagagtgtgactgcactccagggtttcactgcctgggggcaggatgcagcatgtgtgaacaggattgtaaacaaggtcaagaactgacaaaaaaaggttgtaaagactgttgctttgggacatttaacgatcagaaacgtggcatctgtcgaccctggacaaactgttctttggatggaaagtctgtgcttgtgaatgggacgaaggagagggacgtggtctgtggaccatctccagccgacctctctccgggagcatcctctgtgaccccgcctgcccctgcgagagagccaggacactctccgcagatcatctccttctttcttgcgctgacgtcgactgcgttgctcttcctgctgttcttcctcacgctccgtttctctgttgttaaacggggcagaaagaaactcctgtatatattcaaacaaccatttatgagaccagtacaaactactcaagaggaagatggctgtagctgccgatttccagaagaagaagaaggaggatgtgaactgtga

SEQ ID NO: 75 - protein, 255 aa, Homo sapiens
MGNSCYNIVATLLLVLNFERTRSLQDPCSNCPAGTFCDNNRNQICSPCPPNSFSSAGGQRTCDICRQCKGVFRTRKECSSTSNAECDCTPGFHCLGAGCSMCEQDCKQGQELTKKGCKDCCFGTFNDQKRGICRPWTNCSLDGKSVLVNGTKERDVVCGPSPADLSPGASSVTPPAPAREPGHSPQIISFFLALTSTALLFLLFFLTLRFSVVKRGRKKLLYIFKQPFMRPVQTTQEEDGCSCRFPEEEEGGCEL

SEQ ID NO: 76 - DNA, 768 bp, Mus musculus
atgggcaacaactgctataacgtggtggtgattgtgctgctgctggtgggctgcgaaaaagtgggcgcggtgcagaacagctgcgataactgccagccgggcaccttttgccgcaaatataacccggtgtgcaaaagctgcccgccgagcacctttagcagcattggcggccagccgaactgcaacatttgccgcgtgtgcgcgggctattttcgctttaaaaaattttgcagcagcacccataacgcggaatgcgaatgcattgaaggctttcattgcctgggcccgcagtgcacccgctgcgaaaaagattgccgcccgggccaggaactgaccaaacagggctgcaaaacctgcagcctgggcacctttaacgatcagaacggcaccggcgtgtgccgcccgtggaccaactgcagcctggatggccgcagcgtgctgaaaaccggcaccaccgaaaaagatgtggtgtgcggcccgccggtggtgagctttagcccgagcaccaccattagcgtgaccccggaaggcggcccgggcggccatagcctgcaggtgctgaccctgtttctggcgctgaccagcgcgctgctgctggcgctgatttttattaccctgctgtttagcgtgctgaaatggattcgcaaaaaatttccgcatatttttaaacagccgtttaaaaaaaccaccggcgcggcgcaggaagaagatgcgtgcagctgccgctgcccgcaggaagaagaaggcggcggcggcggctatgaactg

SEQ ID NO: 77 - protein, 256 aa, Mus musculus
MGNNCYNVVVIVLLLVGCEKVGAVQNSCDNCQPGTFCRKYNPVCKSCPPSTFSSIGGQPNCNICRVCAGYFRFKKFCSSTHNAECECIEGFHCLGPQCTRCEKDCRPGQELTKQGCKTCSLGTFNDQNGTGVCRPWTNCSLDGRSVLKTGTTEKDVVCGPPVVSFSPSTTISVTPEGGPGGHSLQVLTLFLALTSALLLALIFITLLFSVLKWIRKKFPHIFKQPFKKTTGAAQEEDACSCRCPQEEEGGGGGYEL

SEQ ID NO: 78 - DNA, 831 bp, Homo sapiens
atgtgcgtgggcgcgcgccgcctgggccgcggcccgtgcgcggcgctgctgctgctgggcctgggcctgagcaccgtgaccggcctgcattgcgtgggcgatacctatccgagcaacgatcgctgctgccatgaatgccgcccgggcaacggcatggtgagccgctgcagccgcagccagaacaccgtgtgccgcccgtgcggcccgggcttttataacgatgtggtgagcagcaaaccgtgcaaaccgtgcacctggtgcaacctgcgcagcggcagcgaacgcaaacagctgtgcaccgcgacccaggataccgtgtgccgctgccgcgcgggcacccagccgctggatagctataaaccgggcgtggattgcgcgccgtgcccgccgggccattttagcccgggcgataaccaggcgtgcaaaccgtggaccaactgcaccctggcgggcaaacataccctgcagccggcgagcaacagcagcgatgcgatttgcgaagatcgcgatccgccggcgacccagccgcaggaaacccagggcccgccggcgcgcccgattaccgtgcagccgaccgaagcgtggccgcgcaccagccagggcccgagcacccgcccggtggaagtgccgggcggccgcgcggtggcggcgattctgggcctgggcctggtgctgggcctgctgggcccgctggcgattctgctggcgctgtatctgctgcgccgcgatcagcgcctgccgccggatgcgcataaaccgccgggcggcggcagctttcgcaccccgattcaggaagaacaggcggatgcgcatagcaccctggcgaaaatt

SEQ ID NO: 79 - protein, 277 aa, Homo sapiens
MCVGARRLGRGPCAALLLLGLGLSTVTGLHCVGDTYPSNDRCCHECRPGNGMVSRCSRSQNTVCRPCGPGFYNDVVSSKPCKPCTWCNLRSGSERKQLCTATQDTVCRCRAGTQPLDSYKPGVDCAPCPPGHFSPGDNQACKPWTNCTLAGKHTLQPASNSSDAICEDRDPPATQPQETQGPPARPITVQPTEAWPRTSQGPSTRPVEVPGGRAVAAILGLGLVLGLLGPLAILLALYLLRRDQRLPPDAHKPPGGGSFRTPIQEEQADAHSTLAKI

SEQ ID NO: 80 - DNA, 816 bp, Mus musculus
atgtatgtgtgggtgcagcagccgaccgcgctgctgctgctggcgctgaccctgggcgtgaccgcgcgccgcctgaactgcgtgaaacatacctatccgagcggccataaatgctgccgcgaatgccagccgggccatggcatggtgagccgctgcgatcatacccgcgataccctgtgccatccgtgcgaaaccggcttttataacgaagcggtgaactatgatacctgcaaacagtgcacccagtgcaaccatcgcagcggcagcgaactgaaacagaactgcaccccgacccaggataccgtgtgccgctgccgcccgggcacccagccgcgccaggatagcggctataaactgggcgtggattgcgtgccgtgcccgccgggccattttagcccgggcaacaaccaggcgtgcaaaccgtggaccaactgcaccctgagcggcaaacagacccgccatccggcgagcgatagcctggatgcggtgtgcgaagatcgcagcctgctggcgaccctgctgtgggaaacccagcgcccgacctttcgcccgaccaccgtgcagagcaccaccgtgtggccgcgcaccagcgaactgccgagcccgccgaccctggtgaccccggaaggcccggcgtttgcggtgctgctgggcctgggcctgggcctgctggcgccgctgaccgtgctgctggcgctgtatctgctgcgcaaagcgtggcgcctgccgaacaccccgaaaccgtgctggggcaacagctttcgcaccccgattcaggaagaacataccgatgcgcattttaccctggcgaaaatt

SEQ ID NO: 81 - protein, 272 aa, Mus musculus
MYVWVQQPTALLLLALTLGVTARRLNCVKHTYPSGHKCCRECQPGHGMVSRCDHTRDTLCHPCETGFYNEAVNYDTCKQCTQCNHRSGSELKQNCTPTQDTVCRCRPGTQPRQDSGYKLGVDCVPCPPGHFSPGNNQACKPWTNCTLSGKQTRHPASDSLDAVCEDRSLLATLLWETQRPTFRPTTVQSTTVWPRTSELPSPPTLVTPEGPAFAVLLGLGLGLLAPLTVLLALYLLRKAWRLPNTPKPCWGNSFRTPIQEEHTDAHFTLAKI

SEQ ID NO: 82 - DNA, 597 bp, Homo sapiens
atgaaaagcggcctgtggtatttttttctgttttgcctgcgcattaaagtgctgaccggcgaaattaacggcagcgcgaactatgaaatgtttatttttcataacggcggcgtgcagattctgtgcaaatatccggatattgtgcagcagtttaaaatgcagctgctgaaaggcggccagattctgtgcgatctgaccaaaaccaaaggcagcggcaacaccgtgagcattaaaagcctgaaattttgccatagccagctgagcaacaacagcgtgagcttttttctgtataacctggatcatagccatgcgaactattatttttgcaacctgagcatttttgatccgccgccgtttaaagtgaccctgaccggcggctatctgcatatttatgaaagccagctgtgctgccagctgaaattttggctgccgattggctgcgcggcgtttgtggtggtgtgcattctgggctgcattctgatttgctggctgaccaaaaaaaaatatagcagcagcgtgcatgatccgaacggcgaatatatgtttatgcgcgcggtgaacaccgcgaaaaaaagccgcctgaccgatgtgaccctg

SEQ ID NO: 83 - protein, 199 aa, Homo sapiens
MKSGLWYFFLFCLRIKVLTGEINGSANYEMFIFHNGGVQILCKYPDIVQQFKMQLLKGGQILCDLTKTKGSGNTVSIKSLKFCHSQLSNNSVSFFLYNLDHSHANYYFCNLSIFDPPPFKVTLTGGYLHIYESQLCCQLKFWLPIGCAAFVVVCILGCILICWLTKKKYSSSVHDPNGEYMFMRAVNTAKKSRLTDVTL

SEQ ID NO: 84 - DNA, 600 bp, Mus musculus
atgaaaccgtatttttgccgcgtgtttgtgttttgctttctgattcgcctgctgaccggcgaaattaacggcagcgcggatcatcgcatgtttagctttcataacggcggcgtgcagattagctgcaaatatccggaaaccgtgcagcagctgaaaatgcgcctgtttcgcgaacgcgaagtgctgtgcgaactgaccaaaaccaaaggcagcggcaacgcggtgagcattaaaaacccgatgctgtgcctgtatcatctgagcaacaacagcgtgagcttttttctgaacaacccggatagcagccagggcagctattatttttgcagcctgagcatttttgatccgccgccgtttcaggaacgcaacctgagcggcggctatctgcatatttatgaaagccagctgtgctgccagctgaaactgtggctgccggtgggctgcgcggcgtttgtggtggtgctgctgtttggctgcattctgattatttggtttagcaaaaaaaaatatggcagcagcgtgcatgatccgaacagcgaatatatgtttatggcggcggtgaacaccaacaaaaaaagccgcctggcgggcgtgaccagc

SEQ ID NO: 85 - protein, 200 aa, Mus musculus
MKPYFCRVFVFCFLIRLLTGEINGSADHRMFSFHNGGVQISCKYPETVQQLKMRLFREREVLCELTKTKGSGNAVSIKNPMLCLYHLSNNSVSFFLNNPDSSQGSYYFCSLSIFDPPPFQERNLSGGYLHIYESQLCCQLKLWLPVGCAAFVVVLLFGCILIIWFSKKKYGSSVHDPNSEYMFMAAVNTNKKSRLAGVTS

SEQ ID NO: 86 - DNA, 279 bp, Homo sapiens
atgattcatctgggccatattctgtttctgctgctgctgccggtggcggcggcgcagaccaccccgggcgaacgcagcagcctgccggcgttttatccgggcaccagcggcagctgcagcggctgcggcagcctgagcctgccgctgctggcgggcctggtggcggcggatgcggtggcgagcctgctgattgtgggcgcggtgtttctgtgcgcgcgcccgcgccgcagcccggcgcaggaagatggcaaagtgtatattaacatgccgggccgcggc

SEQ ID NO: 87 - protein, 93 aa, Homo sapiens
MIHLGHILFLLLLPVAAAQTTPGERSSLPAFYPGTSGSCSGCGSLSLPLLAGLVAADAVASLLIVGAVFLCARPRRSPAQEDGKVYINMPGRG

SEQ ID NO: 88 - DNA, 237 bp, Mus musculus
atggatccgccgggctatctgctgtttctgctgctgctgccggtggcggcgagccagaccagcgcgggcagctgcagcggctgcggcaccctgagcctgccgctgctggcgggcctggtggcggcggatgcggtgatgagcctgctgattgtgggcgtggtgtttgtgtgcatgcgcccgcatggccgcccggcgcaggaagatggccgcgtgtatattaacatgccgggccgcggc

SEQ ID NO: 89 - protein, 79 aa, Mus musculus
MDPPGYLLFLLLLPVAASQTSAGSCSGCGTLSLPLLAGLVAADAVMSLLIVGVVFVCMRPHGRPAQEDGRVYINMPGRG

SEQ ID NO: 90 - DNA, 342 bp, Homo sapiens
atggggggacttgaaccctgcagcaggctcctgctcctgcctctcctgctggctgtaagtggtctccgtcctgtccaggcccaggcccagagcgattgcagttgctctacggtgagcccgggcgtgctggcagggatcgtgatgggagacctggtgctgacagtgctcattgccctggccgtgtacttcctgggccggctggtccctcgggggcgaggggctgcggaggcagcgacccggaaacagcgtatcactgagaccgagtcgccttatcaggagctccagggtcagaggtcggatgtctacagcgacctcaacacacagaggccgtattacaaatga

SEQ ID NO: 91 - protein, 113 aa, Homo sapiens
MGGLEPCSRLLLLPLLLAVSGLRPVQAQAQSDCSCSTVSPGVLAGIVMGDLVLTVLIALAVYFLGRLVPRGRGAAEAATRKQRITETESPYQELQGQRSDVYSDLNTQRPYYK

SEQ ID NO: 92 - DNA, 345 bp, Mus musculus
atgggggctctggagccctcctggtgccttctgttccttcctgtcctcctgactgtgggaggattaagtcccgtacaggcccagagtgacactttcccaagatgcgactgttcttccgtgagccctggtgtactggctgggattgttctgggtgacttggtgttgactctgctgattgccctggctgtgtactctctgggccgcctggtctcccgaggtcaagggacagcggaagggacccggaaacaacacattgctgagactgagtcgccttatcaggagcttcagggtcagagaccagaagtatacagtgacctcaacacacagaggcaatattacagatga

SEQ ID NO: 93 - protein, 114 aa, Mus musculus
MGALEPSWCLLFLPVLLTVGGLSPVQAQSDTFPRCDCSSVSPGVLAGIVLGDLVLTLLIALAVYSLGRLVSRGQGTAEGTRKQHIAETESPYQELQGQRPEVYSDLNTQRQYYR

SEQ ID NO: 94 - protein, 164 aa, Homo sapiens
MKWKALFTAAILQAQLPITEAQSFGLLDPKLCYLLDGILFIYGVILTALFLRVKFSRSADAPAYQQGQNQLYNELNLGRREEYDVLDKRRGRDPEMGGKPQRRKNPQEGLYNELQKDKMAEAYSEIGMKGERRRGKGHDGLYQGLSTATKDTYDALHMQALPPR

SEQ ID NO: 95 - DNA, 492 bp, Homo sapiens
atgaagtggaaggcgcttttcaccgcggccatcctgcaggcacagttgccgattacagaggcacagagctttggcctgctggatcccaaactctgctacctgctggatggaatcctcttcatctatggtgtcattctcactgccttgttcctgagagtgaagttcagcaggagcgcagagccccccgcgtaccagcagggccagaaccagctctataacgagctcaatctaggacgaagagaggagtacgatgttttggacaagagacgtggccgggaccctgagatggggggaaagccgagaaggaagaaccctcaggaaggcctgtacaatgaactgcagaaagataagatggcggaggcctacagtgagattgggatgaaaggcgagcgccggaggggcaaggggcacgatggcctttaccagggtctcagtacagccaccaaggacacctacgacgcccttcacatgcaggccctgccccctcgctaa

SEQ ID NO: 96 - protein, 164 aa, Mus musculus
MKWKVSVLACILHVRFPGAEAQSFGLLDPKLCYLLDGILFIYGVIITALYLRAKFSRSAETAANLQDPNQLYNELNLGRREEYDVLEKKRARDPEMGGKQQRRRNPQEGVYNALQKDKMAEAYSEIGTKGERRRGKGHDGLYQGLSTATKDTYDALHMQTLAPR

SEQ ID NO: 97 - DNA, 495 bp, Mus musculus
atgaagtggaaagtgtctgttctcgcctgcatcctccacgtgcggttcccaggagcagaggcacagagctttggtctgctggatcccaaactctgctacttgctagatggaatcctcttcatctacggagtcatcatcacagccctgtacctgagagcaaaattcagcaggagtgcagagactgctgccaacctgcaggaccccaaccagctctacaatgagctcaatctagggcgaagagaggaatatgacgtcttggagaagaagcgggctcgggatccagagatgggaggcaaacagcagaggaggaggaacccccaggaaggcgtatacaatgcactgcagaaagacaagatggcagaagcctacagtgagatcggcacaaaaggcgagaggcggagaggcaaggggcacgatggcctttaccagggtctcagcactgccaccaaggacacctatgatgccctgcatatgcagaccctggcccctcgctaa

SEQ ID NO: 98 - protein, 254 aa, Homo sapiens
MWQLLLPTALLLLVSAGMRTEDLPKAVVFLEPQWYRVLEKDSVTLKCQGAYSPEDNSTQWFHNESLISSQASSYFIDAATVDDSGEYRCQTNLSTLSDPVQLEVHIGWLLLQAPRWVFKEEDPIHLRCHSWKNTALHKVTYLQNGKGRKYFHHNSDFYIPKATLKDSGSYFCRGLFGSKNVSSETVNITITQGLAVSTISSFFPPGYQVSFCLVMVLLFAVDTGLYFSVKTNIRSSTRDWKDHKFKWRKDPQDK

SEQ ID NO: 99 - DNA, 762 bp, Homo sapiens
atgtggcagctgctgctgccgaccgcgctgctgctgctggtgagcgcgggcatgcgcaccgaagatctgccgaaagcggtggtgtttctggaaccgcagtggtatcgcgtgctggaaaaagatagcgtgaccctgaaatgccagggcgcgtatagcccggaagataacagcacccagtggtttcataacgaaagcctgattagcagccaggcgagcagctattttattgatgcggcgaccgtggatgatagcggcgaatatcgctgccagaccaacctgagcaccctgagcgatccggtgcagctggaagtgcatattggctggctgctgctgcaggcgccgcgctgggtgtttaaagaagaagatccgattcatctgcgctgccatagctggaaaaacaccgcgctgcataaagtgacctatctgcagaacggcaaaggccgcaaatattttcatcataacagcgatttttatattccgaaagcgaccctgaaagatagcggcagctatttttgccgcggcctgtttggcagcaaaaacgtgagcagcgaaaccgtgaacattaccattacccagggcctggcggtgagcaccattagcagcttttttccgccgggctatcaggtgagcttttgcctggtgatggtgctgctgtttgcggtggataccggcctgtattttagcgtgaaaaccaacattcgcagcagcacccgcgattggaaagatcataaatttaaatggcgcaaagatccgcaggataaa

SEQ ID NO: 100 - protein, 261 aa, Mus musculus
MFQNAHSGSQWLLPPLTILLLFAFADRQSAALPKAVVKLDPPWIQVLKEDMVTLMCEGTHNPGNSSTQWFHNGRSIRSQVQASYTFKATVNDSGEYRCQMEQTRLSDPVDLGVISDWLLLQTPQRVFLEGETITLRCHSWRNKLLNRISFFHNEKSVRYHHYKSNFSIPKANHSHSGDYYCKGSLGSTQHQSKPVTITVQDPATTSSISLVWYHTAFSLVMCLLFAVDTGLYFYVRRNLQTPREYWRKSLSIRKHQAPQDK

SEQ ID NO: 101 - DNA, 786 bp, Mus musculus
atgtttcagaatgcacactctggaagccaatggctacttccaccactgacaattctgctgctgtttgcttttgcagacaggcagagtgcagctcttccgaaggctgtggtgaaactggaccccccatggatccaggtgctcaaggaagacatggtgacactgatgtgcgaagggacccacaaccctgggaactcttctacccagtggttccacaacgggaggtccatccggagccaggtccaagccagttacacgtttaaggccacagtcaatgacagtggagaatatcggtgtcaaatggagcagacccgcctcagcgaccctgtagatctgggagtgatttctgactggctgctgctccagacccctcagcgggtgtttctggaaggggaaaccatcacgctaaggtgccatagctggaggaacaaactactgaacaggatctcattcttccataatgaaaaatccgtgaggtatcatcactacaaaagtaatttctctatcccaaaagccaaccacagtcacagtggggactactactgcaaaggaagtctaggaagtacacagcaccagtccaagcctgtcaccatcactgtccaagatccagcaactacatcctccatctctctagtctggtaccacactgctttctccctagtgatgtgcctcctgtttgcagtggacacgggcctttatttctacgtacggagaaatcttcaaaccccgagggagtactggaggaagtccctgtcaatcagaaagcaccaggctcctcaagacaagtga

SEQ ID NO: 102 - protein, 216 aa, Homo sapiens
MGWIRGRRSRHSWEMSEFHNYNLDLKKSDFSTRWQKQRCPVVKSKCRENASPFFFCCFIAVAMGIRFIIMVAIWSAVFLNSLFNQEVQIPLTESYCGPCPKNWICYKNNCYQFFDESKNWYESQASCMSQNASLLKVYSKEDQDLLKLVKSYHWMGLVHIPTNGSWQWEDGSILSPNLLTIIEMQKGDCALYASSFKGYIENCSTPNTYICMQRTV

SEQ ID NO: 103 - DNA, 648 bp, Homo sapiens
atgggctggattcgcggccgccgcagccgccatagctgggaaatgagcgaatttcataactataacctggatctgaaaaaaagcgattttagcacccgctggcagaaacagcgctgcccggtggtgaaaagcaaatgccgcgaaaacgcgagcccgttttttttttgctgctttattgcggtggcgatgggcattcgctttattattatggtggcgatttggagcgcggtgtttctgaacagcctgtttaaccaggaagtgcagattccgctgaccgaaagctattgcggcccgtgcccgaaaaactggatttgctataaaaacaactgctatcagttttttgatgaaagcaaaaactggtatgaaagccaggcgagctgcatgagccagaacgcgagcctgctgaaagtgtatagcaaagaagatcaggatctgctgaaactggtgaaaagctatcattggatgggcctggtgcatattccgaccaacggcagctggcagtgggaagatggcagcattctgagcccgaacctgctgaccattattgaaatgcagaaaggcgattgcgcgctgtatgcgagcagctttaaaggctatattgaaaactgcagcaccccgaacacctatatttgcatgcagcgcaccgtg

SEQ ID NO: 104 - protein, 232 aa, Mus musculus
MALIRDRKSHHSEMSKCHNYDLKPAKWDTSQEQQKQRLALTTSQPGENGIIRGRYPIEKLKISPMFVVRVLAIALAIRFTLNTLMWLAIFKETFQPVLCNKEVPVSSREGYCGPCPNNWICHRNNCYQFFNEEKTWNQSQASCLSQNSSLLKIYSKEEQDFLKLVKSYHWMGLVQIPANGSWQWEDGSSLSYNQLTLVEIPKGSCAVYGSSFKAYTEDCANLNTYICMKRAV

SEQ ID NO: 105 - DNA, 696 bp, Mus musculus
atggcgctgattcgcgatcgcaaaagccatcatagcgaaatgagcaaatgccataactatgatctgaaaccggcgaaatgggataccagccaggaacagcagaaacagcgcctggcgctgaccaccagccagccgggcgaaaacggcattattcgcggccgctatccgattgaaaaactgaaaattagcccgatgtttgtggtgcgcgtgctggcgattgcgctggcgattcgctttaccctgaacaccctgatgtggctggcgatttttaaagaaacctttcagccggtgctgtgcaacaaagaagtgccggtgagcagccgcgaaggctattgcggcccgtgcccgaacaactggatttgccatcgcaacaactgctatcagttttttaacgaagaaaaaacctggaaccagagccaggcgagctgcctgagccagaacagcagcctgctgaaaatttatagcaaagaagaacaggattttctgaaactggtgaaaagctatcattggatgggcctggtgcagattccggcgaacggcagctggcagtgggaagatggcagcagcctgagctataaccagctgaccctggtggaaattccgaaaggcagctgcgcggtgtatggcagcagctttaaagcgtataccgaagattgcgcgaacctgaacacctatatttgcatgaaacgcgcggtg

SEQ ID NO: 106 - protein, 4 aa, Artificial sequence
  CD28 YMNM
YMNM

SEQ ID NO: 107 - protein, 4 aa, Artificial sequence
  CD28 PYAP
PYAP

SEQ ID NO: 108 - protein, 4 aa, Artificial sequence
  CD28 FMNM
FMNM

SEQ ID NO: 109 - protein, 4 aa, Artificial sequence
  CD28 AYAA
AYAA

SEQ ID NO: 110 - protein, 21 aa, Artificial sequence
  Signal peptide
ATMGWSCIILFLVATATGVHS

SEQ ID NO: 111 - DNA, 57 bp, Artificial sequence
  Signal peptide DNA sequence
atgggatggagctgtatcatcctcttcttggtagcaacagctaccggtgtgcactcc

SEQ ID NO: 112 - protein, 449 aa, Artificial sequence
  Anti-CD20 (GA101) heavy chain
QVQLVQSGAEVKKPGSSVKVSCKASGYAFSYSWINWVRQAPGQGLEWMGRIFPGDGDTDYNGKFKGRVTITADKSTSTAYMELSSLRSEDTAVYYCARNVFDGYWLVYWGQGTLVTVSSASTKGPSVFPLAPSSKSTSGGTAALGCLVKDYFPEPVTVSWNSGALTSGVHTFPAVLQSSGLYSLSSVVTVPSSSLGTQTYICNVNHKPSNTKVDKKVEPKSCDKTHTCPPCPAPELLGGPSVFLFPPKPKDTLMISRTPEVTCVVVDVSHEDPEVKFNWYVDGVEVHNAKTKPREEQYNSTYRVVSVLTVLHQDWLNGKEYKCKVSNKALPAPIEKTISKAKGQPREPQVYTLPPSRDELTKNQVSLTCLVKGFYPSDIAVEWESNGQPENNYKTTPPVLDSDGSFFLYSKLTVDKSRWQQGNVFSCSVMHEALHNHYTQKSLSLSPGK

SEQ ID NO: 113 - protein, 219 aa, Artificial sequence
  Anti-CD20 (GA101) light chain
DIVMTQTPLSLPVTPGEPASISCRSSKSLLHSNGITYLYWYLQKPGQSPQLLIYQMSNLVSGVPDRFSGSGSGTDFTLKISRVEAEDVGVYYCAQNLELPYTFGGGTKVEIKRTVAAPSVFIFPPSDEQLKSGTASVVCLLNNFYPREAKVQWKVDNALQSGNSQESVTEQDSKDSTYSLSSTLTLSKADYEKHKVYACEVTHQGLSSPVTKSFNRGEC

SEQ ID NO: 114 - protein, 447 aa, Artificial sequence
  Anti-FAP(4B9) PGLALA heavy chain
EVQLLESGGGLVQPGGSLRLSCAASGFTFSSYAMSWVRQAPGKGLEWVSAIIGSGASTYYADSVKGRFTISRDNSKNTLYLQMNSLRAEDTAVYYCAKGWFGGFNYWGQGTLVTVSSASTKGPSVFPLAPSSKSTSGGTAALGCLVKDYFPEPVTVSWNSGALTSGVHTFPAVLQSSGLYSLSSVVTVPSSSLGTQTYICNVNHKPSNTKVDKKVEPKSCDKTHTCPPCPAPEAAGGPSVFLFPPKPKDTLMISRTPEVTCVVVDVSHEDPEVKFNWYVDGVEVHNAKTKPREEQYNSTYRVVSVLTVLHQDWLNGKEYKCKVSNKALGAPIEKTISKAKGQPREPQVYTLPPSRDELTKNQVSLTCLVKGFYPSDIAVEWESNGQPENNYKTTPPVLDSDGSFFLYSKLTVDKSRWQQGNVFSCSVMHEALHNHYTQKSLSLSPGK

SEQ ID NO: 115 - protein, 215 aa, Artificial sequence
  Anti-FAP(4B9) light chain
EIVLTQSPGTLSLSPGERATLSCRASQSVTSSYLAWYQQKPGQAPRLLINVGSRRATGIPDRFSGSGSGTDFTLTISRLEPEDFAVYYCQQGIMLPPTFGQGTKVEIKRTVAAPSVFIFPPSDEQLKSGTASVVCLLNNFYPREAKVQWKVDNALQSGNSQESVTEQDSKDSTYSLSSTLTLSKADYEKHKVYACEVTHQGLSSPVTKSFNRGEC

SEQ ID NO: 116 - protein, 451 aa, Artificial sequence
  Anti-CEA (A5B7) PGLALA heavy chain
EVQLVESGGGLVQPGRSLRLSCAASGFTVSSYWMHWVRQAPGKGLEWVGFIRNKANGGTTEYAASVKGRFTISRDDSKNTLYLQMNSLRAEDTAVYYCARDRGLRFYFDYWGQGTTVTVSSASTKGPSVFPLAPSSKSTSGGTAALGCLVKDYFPEPVTVSWNSGALTSGVHTFPAVLQSSGLYSLSSVVTVPSSSLGTQTYICNVNHKPSNTKVDKKVEPKSCDKTHTCPPCPAPEAAGGPSVFLFPPKPKDTLMISRTPEVTCVVVDVSHEDPEVKFNWYVDGVEVHNAKTKPREEQYNSTYRVVSVLTVLHQDWLNGKEYKCKVSNKALGAPIEKTISKAKGQPREPQVYTLPPSRDELTKNQVSLTCLVKGFYPSDIAVEWESNGQPENNYKTTPPVLDSDGSFFLYSKLTVDKSRWQQGNVFSCSVMHEALHNHYTQKSLSLSPGK

SEQ ID NO: 117 - protein, 223 aa, Artificial sequence
  Anti-CEA (A5B7) light chain
QAVLTQPASLSASPGASASLTCTLRRGINVGAYSIYWYQQKPGSPPQYLLRYKSDSDKQQGSGVSSRFSASKDASANAGILLISGLQSEDEADYYCMIWHSGASAVFGGGTKLTVLRTVAAPSVFIFPPSDEQLKSGTASVVCLLNNFYPREAKVQWKVDNALQSGNSQESVTEQDSKDSTYSLSSTLTLSKADYEKHKVYACEVTHQGLSSPVTKSFNRGEC

SEQ ID NO: 118 - protein, 451 aa, Artificial sequence
  Anti-CEA (T84.66LCHA) PGLALA heavy chain
QVQLVQSGAEVKKPGSSVKVSCKASGFNIKDTYMHWVRQAPGQGLEWMGRIDPANGNSKYVPKFQGRVTITADTSTSTAYMELSSLRSEDTAVYYCAPFGYYVSDYAMAYWGQGTLVTVSSASTKGPSVFPLAPSSKSTSGGTAALGCLVKDYFPEPVTVSWNSGALTSGVHTFPAVLQSSGLYSLSSVVTVPSSSLGTQTYICNVNHKPSNTKVDKKVEPKSCDKTHTCPPCPAPEAAGGPSVFLFPPKPKDTLMISRTPEVTCVVVDVSHEDPEVKFNWYVDGVEVHNAKTKPREEQYNSTYRVVSVLTVLHQDWLNGKEYKCKVSNKALGAPIEKTISKAKGQPREPQVYTLPPSRDELTKNQVSLTCLVKGFYPSDIAVEWESNGQPENNYKTTPPVLDSDGSFFLYSKLTVDKSRWQQGNVFSCSVMHEALHNHYTQKSLSLSPGK

SEQ ID NO: 119 - protein, 218 aa, Artificial sequence
  Anti-CEA (T84.66LCHA) light chain
EIVLTQSPATLSLSPGERATLSCRAGESVDIFGVGFLHWYQQKPGQAPRLLIYRASNRATGIPARFSGSGSGTDFTLTISSLEPEDFAVYYCQQTNEDPYTFGQGTKLEIKRTVAAPSVFIFPPSDEQLKSGTASVVCLLNNFYPREAKVQWKVDNALQSGNSQESVTEQDSKDSTYSLSSTLTLSKADYEKHKVYACEVTHQGLSSPVTKSFNRGEC

SEQ ID NO: 120 - protein, 451 aa, Artificial sequence
  Anti-CEA (CH1A1A98/992F1) PGLALA heavy chain
QVQLVQSGAEVKKPGASVKVSCKASGYTFTEFGMNWVRQAPGQGLEWMGWINTKTGEATYVEEFKGRVTFTTDTSTSTAYMELRSLRSDDTAVYYCARWDFAYYVEAMDYWGQGTTVTVSSASTKGPSVFPLAPSSKSTSGGTAALGCLVKDYFPEPVTVSWNSGALTSGVHTFPAVLQSSGLYSLSSVVTVPSSSLGTQTYICNVNHKPSNTKVDKKVEPKSCDKTHTCPPCPAPEAAGGPSVFLFPPKPKDTLMISRTPEVTCVVVDVSHEDPEVKFNWYVDGVEVHNAKTKPREEQYNSTYRVVSVLTVLHQDWLNGKEYKCKVSNKALGAPIEKTISKAKGQPREPQVCTLPPSRDELTKNQVSLSCAVKGFYPSDIAVEWESNGQPENNYKTTPPVLDSDGSFFLVSKLTVDKSRWQQGNVFSCSVMHEALHNHYTQKSLSLSPGK

SEQ ID NO: 121 - protein, 215 aa, Artificial sequence
  Anti-CEA (CH1A1A98/992F1) light chain
DIQMTQSPSSLSASVGDRVTITCKASAAVGTYVAWYQQKPGKAPKLLIYSASYRKRGVPSRFSGSGSGTDFTLTISSLQPEDFATYYCHQYYTYPLFTFGQGTKLEIKRTVAAPSVFIFPPSDEQLKSGTASVVCLLNNFYPREAKVQWKVDNALQSGNSQESVTEQDSKDSTYSLSSTLTLSKADYEKHKVYACEVTHQGLSSPVTKSFNRGEC

SEQ ID NO: 122 - protein, 449 aa, Artificial sequence
  Anti-CEA (hMN14) PGLALA heavy chain
EVQLVESGGGVVQPGRSLRLSCSASGFDFTTYWMSWVRQAPGKGLEWIGEIHPDSSTINYAPSLKDRFTISRDNAKNTLFLQMDSLRPEDTGVYFCASLYFGFPWFAYWGQGTPVTVSSASTKGPSVFPLAPSSKSTSGGTAALGCLVKDYFPEPVTVSWNSGALTSGVHTFPAVLQSSGLYSLSSVVTVPSSSLGTQTYICNVNHKPSNTKVDKKVEPKSCDKTHTCPPCPAPEAAGGPSVFLFPPKPKDTLMISRTPEVTCVVVDVSHEDPEVKFNWYVDGVEVHNAKTKPREEQYNSTYRVVSVLTVLHQDWLNGKEYKCKVSNKALGAPIEKTISKAKGQPREPQVYTLPPSRDELTKNQVSLTCLVKGFYPSDIAVEWESNGQPENNYKTTPPVLDSDGSFFLYSKLTVDKSRWQQGNVFSCSVMHEALHNHYTQKSLSLSPGK

SEQ ID NO: 123 - protein, 213 aa, Artificial sequence
  Anti-CEA (hMN14) light chain
DIQLTQSPSSLSASVGDRVTITCKASQDVGTSVAWYQQKPGKAPKLLIYWTSTRHTGVPSRFSGSGSGTDFTFTISSLQPEDIATYYCQQYSLYRSFGQGTKVEIKRTVAAPSVFIFPPSDEQLKSGTASVVCLLNNFYPREAKVQWKVDNALQSGNSQESVTEQDSKDSTYSLSSTLTLSKADYEKHKVYACEVTHQGLSSPVTKSFNRGEC

SEQ ID NO: 124 - protein, 451 aa, Artificial sequence
  Anti-TNC (2B10) PGLALA heavy chain
QVQLVQSGAEVKKPGSSVKVSCKASGGTFSSYAISWVRQAPGQGLEWMGGIIPIFGTANYAQKFQGRVTITADKSTSTAYMELSSLRSEDTAVYYCARLYGYAYYGAFDYWGQGTTVTVSSASTKGPSVFPLAPSSKSTSGGTAALGCLVKDYFPEPVTVSWNSGALTSGVHTFPAVLQSSGLYSLSSVVTVPSSSLGTQTYICNVNHKPSNTKVDKKVEPKSCDKTHTCPPCPAPEAAGGPSVFLFPPKPKDTLMISRTPEVTCVVVDVSHEDPEVKFNWYVDGVEVHNAKTKPREEQYNSTYRVVSVLTVLHQDWLNGKEYKCKVSNKALGAPIEKTISKAKGQPREPQVCTLPPSRDELTKNQVSLSCAVKGFYPSDIAVEWESNGQPENNYKTTPPVLDSDGSFFLVSKLTVDKSRWQQGNVFSCSVMHEALHNHYTQKSLSLSPGK

SEQ ID NO: 125 - protein, 214 aa, Artificial sequence
  Anti-TNC (2B10) light chain
DIQMTQSPSSLSASVGDRVTITCRASQGIRNDLGWYQQKPGKAPKRLIYAASSLQSGVPSRFSGSGSGTEFTLTISSLQPEDFATYYCLQNGLQPATFGQGTKVEIKRTVAAPSVFIFPPSDEQLKSGTASVVCLLNNFYPREAKVQWKVDNALQSGNSQESVTEQDSKDSTYSLSSTLTLSKADYEKHKVYACEVTHQGLSSPVTKSFNRGEC

SEQ ID NO: 126 - protein, 449 aa, Artificial sequence
  Anti-HER2 (PER) PG LALA heavy chain 1
EVQLVESGGGLVQPGGSLRLSCAASGFTFTDYTMDWVRQAPGKGLEWVADVNPNSGGSIYNQRFKGRFTLSVDRSKNTLYLQMNSLRAEDTAVYYCARNLGPSFYFDYWGQGTLVTVSSASTKGPSVFPLAPSSKSTSGGTAALGCLVKDYFPEPVTVSWNSGALTSGVHTFPAVLQSSGLYSLSSVVTVPSSSLGTQTYICNVNHKPSNTKVDKKVEPKSCDKTHTCPPCPAPEAAGGPSVFLFPPKPKDTLMISRTPEVTCVVVDVSHEDPEVKFNWYVDGVEVHNAKTKPREEQYNSTYRVVSVLTVLHQDWLNGKEYKCKVSNKALGAPIEKTISKAKGQPREPQVYTLPPSRDELTKNQVSLTCLVKGFYPSDIAVEWESNGQPENNYKTTPPVLDSDGSFFLYSKLTVDKSRWQQGNVFSCSVMHEALHNHYTQKSLSLSPGK

SEQ ID NO: 127 - protein, 214 aa, Artificial sequence
  Anti-HER2 (PER) light chain 1
DIQMTQSPSSLSASVGDRVTITCKASQDVSIGVAWYQQKPGKAPKLLIYSASYRYTGVPSRFSGSGSGTDFTLTISSLQPEDFATYYCQQYYIYPYTFGQGTKVEIKRTVAAPSVFIFPPSDEQLKSGTASVVCLLNNFYPREAKVQWKVDNALQSGNSQESVTEQDSKDSTYSLSSTLTLSKADYEKHKVYACEVTHQGLSSPVTKSFNRGEC

SEQ ID NO: 128 - protein, 449 aa, Artificial sequence; identical to SEQ ID NO: 126
  Anti-HER2 (PER) PG LALA heavy chain 2

SEQ ID NO: 129 - protein, 214 aa, Artificial sequence; identical to SEQ ID NO: 127
  Anti-HER2 (PER) light chain 2

SEQ ID NO: 130 - protein, 330 aa, Homo sapiens [sequence omitted]